European Patent Application EP 4 186 917 A1, published May 31, 2023. Title: Tobamovirus resistant plants. Applicant: Keygene N.V. The sequence listing filed with the application follows.

SEQUENCE LISTING (69 sequences)

SEQ ID NO: 1 - protein, 962 aa, Lycopersicon esculentum
MNDSLAITASSLAITEKKPQRPGGCVGIFFQLFDWNRRFAKKKLFPKKLLSPARLKQASKKFGGDEKQPKHRLIANENSGGFPIAKSNGMSNTRCESKREMKAPSLVARLMGLESMPAGPGSKAKKASASETGSYVAEKLDARPGGSDKEDMDCEKAEIKRELRPQKLQKIGVSERRPVSRFSAEALQLRTVLSRPRKHQPKLTSPVKSPRNVSGRNASRLIGAATRILEPGLQKSRAKCALTYPKYFSPLEDKADLALHHLEVPNPCVDSKTSEVRASVPSCKNCGYMLHSKNGTPNGEEHPSSVSSPVSSYSQPSCQGPGRNMLRLPIINSRDQLERVFEGSSSDANAEIDDVSYCAELILGKRPISRSRIAMHGACQGSNVKKDASSVTHVLNQKQNQTSQNRERGFMKSKQSSLQSNRVLAAAESTINTKSFVAQNRRLGASTRLRMPATADGCKFETERKPYSRRSDSLSPVRKKRLMNVSRQGESSSFVNANLGRESSPYSDKTSRKDVFPISSVNSHSTKPKLPCLRESGATNNSSEGSNVVSFTFRSAMKQKAGIHAEVTKRKSQNSSSFDATPGRSFFTGNDETACLQKSFPLKGDILGALLEQKLKELTSEEEFAEGDAAPRKSTATILQELITALNDETQFHLDSLPSKPNRKEDLYDDREVSSRNTSMNFQAIPDSATDLVGNSLDNDHLSPGCVLEATFSTDSYLSSSPNSSSKDKVLAESVDSIYDEPLFPEPDRDLSDCATSLFTRRSCRALITDHVNNISGVLSKINQLKGSKLGYANEVILNTELILGTSPEQQALPVDDGLSVSHFLLNELEMLSSLLWMTFGQLLGCNDPKQMNQLKGFAFDCLLEYLDSKFGRYSDSGFRIWSKLPSSMTKEILIADIIEEVKEWTEFVGLIPDELIEWDMSHSLGKWTDFEIEEFECGTEVDRHILQVLVDEVVLDLYSSS

SEQ ID NO: 2 - protein, 556 aa, Lycopersicon esculentum
MMAGEKIIEKPEAVAPGLKSDPSNKLIEKDLVSKKDGKAADSVASLGAVTSIKCENDQPPAAEQGYNGTYNQLDEQAYFNAGVQSDNGSLLYYMPGYNPYSAGFVGGDGKQPYPSSGYLQQPVSYGSDSMPCYTWGSPYCADITNSAAPKSGNVKSTFGRNGSVKSNGFNSTKTNSSFSSKNSTVLFNPKSRPATAMSNPPKSFHQAQPFNPVNKFQSDVQSGGLMKGFHLVGDYPSYTSQNQGFFMPYDPINCQTNSRMWNGNYRAKPRGNFTRNGVFEATNELPRGPRANGRSVPSKPSAEEDQLVPAVQREKYNKEDFKTQYDNAKFYIIKSYSEDDIHKCVKYDVWSSTPNGNKKLDTAFVESEAKASGTGSSCPVFLFFSVNGSGQFLGVAEMVGQVDFNRNMDFWQLDKWSGFFPLKWHIVKDVPNTQFRHIILENNDNRPVTYSRDTQEIGLKEGLEMLNILKNYSEKTSILDDFNFYEKREKVLKAKRSSKPVIQADAYEKADSLKQFKGGDKVLEEELKTNSTDPTAPLVSLTKNLSINSRPFKSSV

SEQ ID NO: 3 - protein, 471 aa, Lycopersicon esculentum
MDEKLIQRLESAVSRLEALSVGGGVSLGDGEAAAALDPSIIAFDDLRSRFVGRVCTAAEKIGGQVLDVTKIVEEAFEAQRELLIKIKETQKPSMSGLAEFLKPLNDVIVKGTKMTEGRRSDLFNHLKAAVDSLTALAWIAYTGKDCGMSMPIAHVEESWQMAEFYNNKVLVEFRNKDPDHVEWAKALKEIYLPGLRDYVKSHYPLGPAWSATGKVAVSAPPKAPAPSRPMPPPLPPASLFSSESPQASSSRPKKGMSAVFDEINSGKPVTGGLRKVTDDMKTKNRADRTGVISAGEKERRVSSPSFSKAGPPKLELQMGRKWVVENQIGRKNLVIDDCDAKQSVYIFGCKDSVLQIQGKVNNITIDKCTKMGVVFSDVVAACEVVNCNGVEVQCQGSAPTISVDNTTGCQLYLSKDSLGTSITTAKSSEINVLVPGAGADSDWGEHALPQQFSHVYKSGQFVTTPVSHSGG

SEQ ID NO: 4 - protein, 494 aa, Lycopersicon esculentum
MAAIAPEVGEEREIQKSYWMEQTSELNLEAMMRDSAASDLDKEDRPEVLSLLPSYEGKSVLELGAGIGRFTGDLAEKAGELVAVDFIEEVTKKNESINGHHKNVKFVCADVTSPDLTVLPESVDLIFSNWLLMYLSNEEVQDLAERMIKWLKVGGYIFFRETCFHQSGDHKGKNNPTHYREPRFYTKVFQECTLKDDAGKSYELSLIGYKCIETYVKNKKNQNEICWIWQKVHSEDDRGFQHFLDTVQYKSNGILRYERVFGAGFVSTGGIDTTKEFVAMMDLQPGEKVLDVGCGIGGGDFYMAEKYDVHVVGIDLSVNMITLAFERAIGRKCAVEFEVADCTVKTYPEESFDVIYSRDTILHIQDKPALFRSFYKWLKPGGRVLISDYCKKAGPASEDFAAYIKQRGYDLHDVEAYGQMLRDAGFNEVIADDRTEQFMQVLQKELDTVENERELFIQEFSEQDYNDIVGGWKAKLVRSSSGEQRWGLFFAKKN

SEQ ID NO: 5 - protein, 508 aa, Lycopersicon esculentum
MECNKDEAFRAKKIAERKFEQKDYAGAKKFALKAQVLYPGLDDLTQMLTTFDVYISAENKVSGEVDWYGVLGVSPSSDDETVKKQYRKLALVLHPDKNKSIGAEGAFQLLSEAWSLLSDKSKRLAYNQRRSSKGPQQKQQKVPVPSGGPSTFWTICHRCKMHYEYLKIYLNHTLLCPNCHESTSQWKRERRLKGVKKVPDPDFHNFDQDRSESCFEDNEVWASYDADDGMPRFYALINKVISREPFKVRLSWLNSKTNTEFGPMEWVASGFYKTSGEFRIGRYETGKSVNSFSHKVRWSKGPRGTVLIYPQKGDVWALFRNWSADWNQNTPDDVIHKYDMVLVLDDYNEEQGISVAPLIKVAGFKTVFRPDLNPEKMIRITREEMFRFSHQVPSHLLTGEEGQNAPKGCQELDPAATPLELLQTVTETNEVPAMQNDKEANGGSSQKVQETKTSEAADHTLKSREGGMVESEGEISLGSEQMVEKVTMEQTQVNPVKTDKATKFGTET

SEQ ID NO: 6 - protein, 413 aa, Lycopersicon esculentum
MALILHSTDNNKNASKALIAAEYTGVKVDLAKDFQMGVSNKTPEFLEMNPIGKVPVLQTPDGPVFESNAIARYVTKTKPNNPLFGSSLIEYAQIEQWNDFSATEIDANIARWLYPRLGYAVYISQAEEGAVAALKRALGALNTHLASNTYLVGHFITLADIIMVCNLSIGFRMILTKSFTKEFPHVERYFWTVVNQPNFVKILGEVKQAESIPAVQSKPAQPEKLKAKEEPKKEVKKEEPSPVEEEAAPKPKAKNPLDLLPPSKMILDDWKRLYSNTKTNFREVAVKGFWDMYDPEGYSLWFCDYKYNDENTVSFVTLNKVGGFLQRMELVRKYAFGKMLIVGSEAPFKVQGLWLFRGKEIPKFVMEEVYDMELYEWKEVDINDEAQKERVSQMIEDHEPFEGQALLDAKCFK

SEQ ID NO: 7 - protein, 1924 aa, Lycopersicon esculentum
MAPNKNGRGKTKGDKKKKEEKVLPVVMDITINLPEETQVILKGISTDRIIDVRRLLSVNTTTCNVTNFSLSHELRGPRLKETVDVSALKPCILTLIEEEYDEESATAHVRRLLDIVACTTSFGPSGTSGKELKTDSCKNARGVQDNKNAKKSNKVRGNDKSSSPPQTPTPVAQQLGKDAGSEEVDGEMSNTCPKIGSFYEFFSLSHLTPPLQCNAPSLSHIVSLFSCFLLKLRLILILAVIRRATRQQDDEVLPDDHLFSLEVKLCNGKLVIVEACKKGFYNFGKQGILCHNLVDLLRQLSRAFDNAYDDLMKAFLERNKFGNLPYGFRANTWLIPPVAAQLPAIFPPLPVEDDTWGANGGGLGRDGKFDSLPFANEFLNVASMACKTTEERQIRDRKAFILHSLFVDVAILRAISAVKHVMEKVKPAHCDLNGEIIYNETVGDLSIFVTKDSSNASCKVDTKIDGFQATGIAMKNLMERNLLKGITADENTAAHDIATLGVLNVRHCGYIATVKVQGKENDKVGSPLQSMELADQPDGGANALNINSLRLLLHKKVDNKVMHSKPSETEEPNCSQAFVRRILEESLTKLEEEKIEGDSFIRWELGACWIQHLQDQKKSEKDKKPSAEKKKNEMKVEGLGIPLKSLKNRKKSTDGTNMESQSESFKSAADGVGGGSEKPVLQSGESQFETDTDQNQVVLKALLSDAGFTRLKESETGLHLKSLEELIDLSQKYYNEVALPKLVADFGSLELSPVDGRTLTDFMHTRGLRMRSLGQVVKLSEKLSHVQSLCIHEMIVRAFKHILQAAIASVVDIEDIAAIIAAALNMMLGVPENDDSNEYGVDSLIWRWLKLFLKKRYEWDVGSLNYKDMRKFAILRGLCHKVGIELVPRDYDMSSASPFQKVDIVSLVPVHKQAACSSADGRQLLESSKTALDKGKLEDAVSYGTKALAKLVAVCGPYHRMTAGAYSLLAVVLYHTGDFNQATIYQQKALDINERELGLDHPDTMKSYGDLAVFYYRLQHTELALKYVKRALYLLHLTCGPSHPNTAATYINVAMMEEGLGNVHVALRYLHKALKCNQKLLGPDHIQTAASYHAIAIALSLMEAYPLSVQHEQTTLQILRAKLGPDDLRTQDAAAWLEYFESKAFEQQEAARNGTKKPDASIASKGHLSVSDLLDYINPSPDAKGRDVGSKRRGFVSKALISQVKGKSDQNNVAIPNSDTFKDVPKEETDEKKQIVEDHTDPKMNMEPVDTVIESHHNGDGGITENKPIQSGPLLKETSIEKSMVREVLSEPSAEAEDGWQPVQRPRSGGFYGRRRRQRRQTISKVIGYQKKDPISDVDHAKLKNNYQASKYYVLKKRTSPGSYADYYLAKSQASGTKLGRRVIKAVAYRVKSVSSSVRDAVPEISTTGGDLLNTSSEQVQVSATKEVGSLSKRSSIVNLGKSPSYKEVALAPPGTISMLQERVSEDEIPDNPDVMKLEKESNGAEENSKIMGRDAESMEKENIQDLVANSSDHVKSETVDTDSKEEIQMSDLKGGEISDLISANASIQPGHVDVSPMEQGSVKTHNVPTSDNSPKADPCEKDSSSNLNPGVISNMTLQDMDHLKVKSASSHASDASRELSRKLSASAAPFSPSPAVPRGTPLPMNINLPSPPGTRPPIGPWSVTMSLHQGPPTILPSPMCSSPHHLYPSPPHTPNMMHPLRFIYPPYSQPQTLPPNTFPMSSSTFHPNHYAWQCNIAPNASEYVPATVWPGCHPVEFSISPPVIEPITDSISSAKEISDNPENITLTTSLLVDLNTGDEVKEDVNLPASETVENIAAVVPEKERASNTPDSHFVTSSSDQSKEGSGSNHVQRNLTETDNEKTFNILVRGRRNRKQTLRMPISLLKRPYSSQPFKAVYSRVIRETEVPSSTSFDPHEHGITTAT

SEQ ID NO: 8 - protein, 250 aa, Lycopersicon esculentum
MGDLHSIAYNSFSSLGCDFHGLEVLNNDMSPFMESTPPFLSNFDCELSSGYLQDALFKFNSKRRRLFLFNDDDDKENYQNKDSIKNLWSSTIDQQFSEDYDSFSQITKCDSFSGDPMSKMSEEYSKRTEEEAISENYYYSSNSSPTSSSHHNKQPLQYGGGDKKRRMCGKIVYPFGLVKPGGQEGDVTLNDINERILMRPTRPVRHPVGDFACRSTVCPAGPGLSGKTVVALTKIHTQGRGTITIIRTRG

SEQ ID NO: 9 - protein, 969 aa, Capsicum annuum
MNVSSAREMNDSLAITASSLAITEKKPQRPGGCVGIFFQLFDWNRRFAKKKLFPKKLLSPDRLKQASKKFGGDEKQPKIRLIANENSGGFPNVKNNGMTNTCCESKRKMKAPSLVARLMGLESMPAASGSKPKKASGSEIGSNVAEKLGGQPGGSDKEDMDFEKAEIKRELRPQKLQKIGLSERRSVCRFSAEALQLRTVLSRPRKHQPKLVSPVKSPRNVSGRNASRLIGAATRILEPGLQKSRVKCALTYPTRYFSPLEDKADLAPHHLEGPNPCVDSKTLKGTSVPSCKNCGYFLHSKNGIPNVEEHSSSVSSPISSYSGPPCHGPGRNIPKLPIFSSRDQLERVSEGSSSDATAEIDDVSYCAELILGKRSISRSRMEMHGTRQGNNVKKDASPVTHVLNQKQNQTSQNRERGLMKSKPSSLQSNRILAAAESMNNTKNFVAQNRRLGASTRLRMPATADGCKFETERKPYSSRSDSFSPVRKKRLNNVSRQGDSSSFVNANMGGESSPSSDKTSRKDVAFPICSVDSHSTKPKLPCLREGVTTNNSSEGCNVVSFTFKSAMKQKAGTHAEVTKRKSQNYSSVDATRGRSFFKGNDEAPCLHKSFPLKGDILGALLEQKLKELTSEEEFGEGGAAPRKSTATILQELITALNEEKQFHLDSSPVRPSRKEDLCDDGDVSSRNTCMNFQAIPDSAATDLVGNSLDHHSPGCVLEAAFSTDSYLSSSPNSSSKDKVLAGSVDSIDDEPLFPEPDRDLSDCETSLSTRSCRALITDHFNNVSGLLSKIDQLKGSKLSYAKEVILNTELIFRTTPQQQALPVEDGFSVSHFLLNELEMLSSLLWMTFSQLLGCNDPKQMNQLKGFAFDCLLEYLDSKFARYSDSGFRTWTKLPSSMTKEILIADIIEEVKEWTEFVGLIPDELIEWDMSHSLGKWTDFEIEEFECGTEVARHILQELVDEVVLDLYSFS

SEQ ID NO: 10 - protein, 569 aa, Capsicum annuum
MAGEKIIEKSEAVAPGLKSDSSTKLTEKDLVSKNDGKVSDSVSSLGAVTGIKGEIDQPPVAEQGAYYPPTSYCDYYYPGYNGTYNQLDDQAYFNSGVQSENGSLLYYMPGYNPYGAGYIGGDGKQPYLSSGYLQQPVSYGSDSMPCYSWGGSTYCADITNSAAPKSGNVKSTFGRNGSVRSNGFNPTKTNGSFSSKNSTMLFNPKNRPSTAISNPPKSIHQAQPFNPANKSDVQSGGLTKGYHMVGDFPSYSSQNQGFFMPYDPIHYQTNSRLWNGNYRGKPRGNFTRNGVFEASNELPRGPRANSRSAPSKPSAEEDQLEPTIQREKYNKEDFKTQYDNAKFYIIKSYSEDDIHKCVKYAVWSSTPNGNKKLDTAFLDAEGKASGTDSSCPVFLFFSVNGSGQFLGVAEMVGQVDFNRNMDFWQLDKWSGFFPVKWHIVKDVPNTQFRHIILKNNDNRPVTYSRDTQEIGLKEGLEMLNILKNYSEKTSILDDFNFYEKREKVLKAKRSSKPAIQADVFEKADSVRQFKGGDKVREEELKSNSTDPTASLVSLAKNLSINSRPFKSSV

SEQ ID NO: 11 - protein, 475 aa, Capsicum annuum
MEEKLVQRLESAVARLEALSATGFRSGGSVVAGGDGTAVLDPSIIAFDDLRSQFLSKVLSAAEKIGGQVLDVSKIVEEAFEAQRELLIKIKETKKPDNSGLVEFLKPLNDVIVKATKMTEGRRSDFFNHLKSAVDSLSALAWIAYIGKDCGMSMPIAFVEESWQMAEFYNNKILVEFKNKDPNHVEWAKALKELYLPGLRDYVKSHYPLGPVWSATGKPAVSAPSKAPSPSAPAPPVPPPASLFSSESPQASSSRPKQGMSAVFDEINSGKPVTSGLRKVTDDMKTKNRFDRTGVVNAGDKEARMSSPPVSKTGPPKLELQMGRKWVVENQVGQKNLVIDDCDTKQSVYVYGCKDSVLQIKGKVNNLTIDKCTKMGIVFAGVVAACEVVNCNSVEVQCQGSAPTISIDNTNGCQLYLNKDSLEGSITTAKSSEINVLVPGAGPDDDWGEHALPQQYAHEYKDGHFVTTPVSHSGA

SEQ ID NO: 12 - protein, 472 aa, Capsicum annuum
MDEKLIQRLESAVIRLEALSVGGGASVGDGVAAAALDPSIIAFDDLRSQFVGRVLGAAEKIGGQVLDVTKIVEEAFEAQRELLIKIKETQKPSMSGLPEFLKPLNDVILKATKMTEGWRLDFFNHLKSAVDSLIALAWIAYTGKDCGMSMPIAHVEESWQMAEFYNNKVLVEFRNKDPNHIEWAKALKELYLPGLWDYVKSHYPLGPVWSATGKVAVSAPSKAPLPTSRPMPPPLPPASLFSSGSFQASSSRPKKGMAAVFDEINSGKPVTTGLRKVTDDMKTKNRADRTGVISAGEKEGRLSSPSFSKAGPPKLELQMGRKWMVENQIGRKNLVIDDCDAKQSVYIFGCKDSVLQIQGKVNNITIDKCTKMGVVFTDVVAACEVVNCNGVEMQCQGSAPTISVDNTTGCQLYLGKDSSETSITTAKSSEINVLVPGAGPDSDWGEHALPQQFSHVYKNGQFVTTSVSHSGG

SEQ ID NO: 13 - protein, 489 aa, Capsicum annuum
MAPGIGQEREIQKSYWIEKTAGLKLEAMMHVHDLESSDLDKEDRHEVLSLLPSYEGKSVLELGAGIGRFTGDLAKKAGELVAVDFIEGVIKENESISGHHKNVKFKCADVTSPDLTFSPESVDLIFSNWLLMYLSDEEVQDLAERMMTWLKVGGYIFFRETCFHQSGDNKGKNNPTHYREPRFYTKVFQECNAGKSYELSLVGYKCMETYVRNKRNQNEICWIWQKVRSDDDRGFQHFLDTVQYKSNGILRYERVFGKDFVSTGGIDTTKEFVAMLDLQPGEKVLDVGCGIGGGDFYMAEKYDVHVLGIDLSVNMISLSFERAIGRKCAVEFEVADCTVKTYPEGSFDVIYSRDTILHIQDKPALFQSFYKWLKPGGRVLISDYCKKAGPASEEFAAYIKQRGYDLHDVEAYGQMLRDAGFNEVIAEDRTELFMKVLQKELDIVEKERESFIQEFSEQDYNDIVGGWKAKLVRSSSGEQRWGLFIAKKN

SEQ ID NO: 14 - protein, 491 aa, Capsicum annuum
MDVASGQEREVQKSYWIEHTAELTVEAMMLDSKAADLDKEERPEVLSLLPAYEGKTVLELGAGIGRFTGELAKKAGQLIALDFIEGAIKKNESINGCHKNVKFMCADVTSPDLNFSPESVDLIFSNWLLMYLSDEEVQDLAKRMVKWLKVGGYIFFRESCFHQSGDHKRKNNPTHYRDPSFYTKVFRECHVNAGDGKSFELSLGGCKCIGAYVRNKKNQNQICWSWQKVGSENDMEFQRFLDTVQYKCSGILRYERVFGQGFVSTGGLETTKEFVAMLDLQPGQKVLDVGCGIGGGDFYMAEKYDVHVVGIDLSINMISFALERAIGLKCAVEFEVADCTKKTYPVGTFDVIYSRDTILHIQDKPALFRSFYKWLKPGGKVLISDYCKRAGPASEEFAGYIKQRGYDLHDVEAYGQMLRDAGFHDVVAEDRTEQFIGVLQKELDTVEKGRESFIHEFSEQDYNEIVGGWKAKLIRSSSGEQRWGLFVAKKN

SEQ ID NO: 15 - protein, 271 aa, Capsicum annuum
MLCWLWQKVNSEDDRGFQRFLDNAQYKCSGILRYERVFGEGYVSTGGIDTTKEFVSMLDLQPGQKVLDVGCGIGGGDFYMAENYDVHVVPIDLSINMISFALERAIGLKCAVKFEVADCTKKTYPDGTFDVIYSRDTILHIQDKLALFRSFYRWLKPGGKVLISDYCKRPGPASEDFSGYIKRRGYDLHYVEAYGLMLREAGFDEVIAKDRTEQFINVLRKELYTVEKERDSFFQEFSEQGYNEIVGGWNAKLLRSSSGEQRWGLFIAKKK

SEQ ID NO: 16 - protein, 730 aa, Capsicum annuum
MECNKDEALRAKIIAERKFEQKDYAGAKKFALKAQALYPGLDALAQMLTTLDIYIAAENKISGEVDWYGVLGVSPSTDDETVRKQYRKLALILHPDKNKSVGAEGAFKLLSEAWSLLSDKSKRLAYNQRRSSKGFQQKAPVHSGGPSAPPRNGFHNFTSKTSKTQKNASRVPSSSVNSSANQRSDTFWTICHRCKMHYEYLKIYLNHTLLCPNCHEAFMATETAPPFNHAKSSNSTRQWHQNAGNHAPNGNQFPIGRNASAGKTSGSAPASSNTANYSNFQQDSFSRMAGVGSSDPSIAAKAANVVQQAHEKMKRERDDSQTRQPPLKQRKLDDNGIRYGSNIPHYAERAYGFSSSKFNSTRELTPLENRNMLMGKARKEILSKLNEWRSQPQDAQKNKVKEGKKEKQRAANVLGQNVNGNVESSAMKGVKKDVNASANDAKQEDLLPQSMNVPDPDFHNFDQDRSESCFGDNEVWAAYDADDGMPRFYALISKVVSREPFKVRLSWLNSKTNSEFGPMEWVASGFYKTSGEFRIGRYETSKSVNSFSHKVRWSKGPRGSVLIFPMKGEVWALYRHWSPDWNQNTPDDVIHKYDMVLVLDDYNEEQGISVAPLVKVAGFKTVFRPDLNSEKVMRITREEMFRFSHRVPSHLLTGEEAQNAPKGCQELDPAATPLELLQTLPETNGVSAMQNDKDFNGLSPQNVQETKTRETADHTLNSSEDGMVNGEEAP

SEQ ID NO: 17 - protein, 414 aa, Capsicum annuum
MALILHSTSNNKNAAKGLIAAEYTGVKVELAKDFQMGVSNKTPEFLEMNPIGKVPVLQTPDGPVFESNAIARYVTKTKPDNLLFGSSLIEYAQIEQWNDFSATEVDANIARWLYPRLGYAVYIPPAEEAAVAALKRALGALNTHLASNTYLVGHSITLADIIMVCNLSIGFGVIMTKSFTKEFPHVERYFWTVVNQPNFCKILGEVKQAESIPAPPSKKPAPATEKPKAKEEPKKEVKEEPKPAEEEAAPKPKPKNPLDLLPPSPMILDDWKRLYSNTKTNFREVAVKGFWDMYDPEGYSLWFCDYKYNDENTVSFVTLNKVGGFLQRMDLVRKYAFGKMLIVGSEPPFKVQGLWLFRGKEIPKFVMDEVYDMELYEWKQVDINDEAQKERVSQMIEDHEPFEGQALLDAKCFK

SEQ ID NO: 18 - protein, 1907 aa, Capsicum annuum
MAPSKNGRGKTKGDKKKKEEKVLPVVMDITINLPDETQVILKGISTDRIIDVRRLLSVNTTTCNITNFSLSHELRGPRLKETVDVSALKPCLLTLIEEDYDEESATAHVIRLLDIVACTTSFGPSGTNGKDLKTESSKNARGAQDSKGAKKSSKVQANDKSSSPPQTPTPAAASQQAGKDAASVDVDGEMSNTCPKIGSFYEFFSLSHLTPPLQFIRRATRQQDGEVLPDDHLFTLEVKLCNGKLVIVEACKKGFYNFGKQGILCHNLVDLLRQVSRAFDNAYDELMKAFSERNKFGNLPYGFRANTWLIPPVAAQLPAIFPPLPVEDENWGANGGGLGRDGKFDLLPYANEFLNVASMPCKTTEERQIRDRKAFLLHSLFVDVAILRAISAVKHVMEKVKPAHCNSNGEIILTESVGDLSIFVTKDASNASSKVDTKIDGFQATGIAMKNLMERNLLKGITADENTAAHDVATLGVLNVRHCGYIATVKVQGKENDKVGSPLQSMELPDQPDGGANALNINSLRLLLHKKVVNKVMHSKPSDSEETNCSQAFVKRILEESLTKLEEEKIEGDSFIRWELGACWIQHLQDQKKSEKDKKNPVEKTKNEMKVEGLGIPLKSLKNRKKSSDGANTESQSDTFKSIADGVQRGSEKTVLQSGESQFETDTDQNQVVLKALLSDAGFTRLKESETGLHLKSLEELIVLSQKYYNEVALPKLVADFGSLELSPVDGRTLTDFMHTRGLRMRSLGQVVKLSEKLSHVQSLCIHEMIVRAFKHILQAVIASVVDIEDMAAIIAAALNMMLGVPENDDANELGVDSLIWIWLELFLKKRYEWDVGSLNYKDVRKFAILRGLCHKVGIELVPRDYDMSSPSPFQKVDIVSLVPVHKQAACSSADGRQLLESSKTALDKGKLEDAVSYGTKALAKLVAVCGPYHRMTAGAYSLLAVVLYHTGDFNQATIYQQKALDINERELGLDHPDTMKSYGDLAVFYYRLQHTELALKYVKRALYLLHLTCGPSHPNTAATYINVAMMEEGLGNVHVALRYLHKALKCNQKLLGPDHIQTAASYHAIAIALSLMEAYPLSVQHEQTTLQILRAKLGPDDLRTQDAAAWLEYFESKAFEQQEAARNGTKKPDASIASKGHLSVSDLLDYINPSPDAKGRDVGSKRKGFVSKALFSQVKGKSEQSNVSIPNSDTPKDVPKEETDEKKQLIEDHTDPKMHMEPVDTVIESNHNGDGRIAENKPIQSGPLLKETLIEKSTVHEVLSEPSAEAEDGWQPVQRPRSGGFYGRRRRQRRQTISKVIGYQKKDPVSDVDHAKLKNNYQASKYYVLKKRTSPGSYADYYIAKSQTPGTKLGRRVIKAVAYRVKSVSPSVRDAVPEISTTGGDLTTSSEQVQVSVTKEVGSVAKRSSIVNLGKSPSYKEVALAPPGTISMLQERVSEGEIPDNQDITKLEEESNGAETNSKTMKSDAESVEKENIQDLVADSADHVKSETVATDKKEEIQMSDLDGGEISDVISANTSIQPGHVDVSPVEQVSVETHNVPPSDNSPKVDPCEKDSSSHLNPTCISNMTLQDMDHLKVKSASSHTSDASRELSRKLSASATPFSPSPAVPRVAPLPMNINLPSPPGIRPPVGPWPVNMSLHQGPPTILPNPMCSSPHHLYPSPPHTPNMMHPLRFIYPPYSQPQTIPPSTFPMNSSTFHPNHYAWQCNIAPNASEYVPATVWPGCHPVEFSISPPVIESITDSISAAKELSDNPESISLTTSLPVDLNTGDEVKEDENLPVSEMVESLAAVGSEKERASNTSDSHFVTFSSDQSKEGSGSNEKAGSCSDNYVQRNLVETDDEKTFNILVRGRRNRKQTLRMPISLLKRPYSSQPFKAVYSRVIRETEVPRSTSFDPHEHCITTAT

SEQ ID NO: 19 - protein, 263 aa, Capsicum annuum
MGDLHSIAYNNNNLHSLSSLGCDFHGLEVFNNDISPFMESTPPFLSNLDCDLSSGYLQDALFKFNSKRRRLLLFDDDDEEKENYQINDSNNSIKNLWSSTMDQQFSEDYDCFSQITKCDSFSGDPMSKMSEEYSKEEAISENYYYYSSSPTSSSHHNNINQKQLPQQYGGVDQKRSKKRMVGKIVCPFGLVKPGGQEGDVTLNDINERILMRPTRPVRHPVGDFACRPTVSPAGPGLSGKKVVALTKIHTQGRGTITIIRTRG

SEQ ID NO: 20 - DNA, 13452 bp, Artificial Sequence
  pJL462 plasmid
gagatggtcacagcttgtctgtaagcggatgccgggagcagacaagcccgtcagggcgcgtcagcgggtgttggcgggtgtcggggcgcagccatgacccagtcacgtagcgatagcggagtgtatactggcttaactatgcggcatcagagcagattgtactgagagtgcaccatatgcggtgtgaaataccgcacagatgcgtaaggagaaaataccgcatcaggcgctcttccgcttcctcgctcactgactcgctgcgctcggtcgttcggctgcggcgagcggtatcagctcactcaaaggcggtaatacggttatccacagaatcaggggataacgcaggaaagaacatgtgagcaaaaggccagcaaaaggccaggaaccgtaaaaaggccgcgttgctggcgtttttccataggctccgcccccctgacgagcatcacaaaaatcgacgctcaagtcagaggtggcgaaacccgacaggactataaagataccaggcgtttccccctggaagctccctcgtgcgctctcctgttccgaccctgccgcttaccggatacctgtccgcctttctcccttcgggaagcgtggcgctttctcatagctcacgctgtaggtatctcagttcggtgtaggtcgttcgctccaagctgggctgtgtgcacgaaccccccgttcagcccgaccgctgcgccttatccggtaactatcgtcttgagtccaacccggtaagacacgacttatcgccactggcagcagccactggtaacaggattagcagagcgaggtatgtaggcggtgctacagagttcttgaagtggtggcctaactacggctacactagaaggacagtatttggtatctgcgctctgctgaagccagttaccttcggaaaaagagttggtagctcttgatccggcaaacaaaccaccgctggtagcggtggtttttttgtttgcaagcagcagattacgcgcagaaaaaaaggatctcaagaagatcctttgatcttttctacggggtctgacgctcagtggaacgaaaactcacgttaagggattttggtcatgcatgatatatctcccaatttgtgtagggcttattatgcacgcttaaaaataataaaagcagacttgacctgatagtttggctgtgagcaattatgtgcttagtgcatctaatcgcttgagttaacgccggcgaagcggcgtcggcttgaacgaatttctagctagacaaggtactaaaacaattcatccagtaaaatataatattttattttctcccaatcaggcttgatccccagtaagtcaaaaaatagctcgacatactgttcttccccgatatcctccctgatcgaccggacgcagaaggcaatgtcataccacttgtccgccctgccgcttctcccaagatcaataaagccacttactttgccatctttcacaaagatgttgctgtctcccaggtcgccgtgggaaaagacaagttcctcttcgggcttttccgtctttaaaaaatcatacagctcgcgcggatctttaaatggagtgtcttcttcccagttttcgcaatccacatcggccagatcgttattcagtaagtaatccaattcggctaagcggctgtctaagctattcgtatagggacaatccgatatgtcgatggagtgaaagagcctgatgcactccgcatacagctcgataatcttttcagggctttgttcatcttcatactcttccgagcaaaggacgccatcggcctcactcatgagcagattgctccagccatcatgccgttcaaagtgcaggacctttggaacaggcagctttccttccagccatagcatcatgtccttttcccgttccacatcataggtggtccctttataccggctgtccgtcatttttaaatataggttttcattttctcccaccagcttatataccttagcaggagacattccttccgtatcttttacgcagcggtatttttcgatcagttttttcaattccggtgatattctcattttagccataacaagaagccatgaaaaccgccactgcgccgttaccaccgctgcgttcggtcaaggttctggaccagttgcgtgacggcagttacgctacttgcattacagcttacgaaccgaacgaggcttatgtccactgggttcgtgcccgaattgatcacaggcagcaacgctctgtcatcgttacaatcaacatgctaccctccgcgagatcatccgtgtttcaaacccggcagcttagttgccgttcttccgaatagcatcggtaacatgagcaaagtctgccgccttacaacggctctcccgctgacgccgtcccggactgatgggctgcctgtatcgagtggtgattttgtgccgagctgccggtcggggagctgttggctggctggtggcaggatatattgtggtgtaaacaaattgacgcttagacaacttaataacacattgcggacgtttttaatgtactgaattaacgccgaattgaattatcagcttgcatgcagctctcccatatggtcgactagaggcctctagggccgttttacgtttggaactgacagaaccgcaacgttgaaggagccactcagccgcgggtttctggagtttaatgagctaagcacatacgtcagaaaccattattgcgcgttcaaaagtcgcctaaggtcactatcagctagcaaatatttcttgtcaaaaatgctccactgacgttccataaattcccctcggtatccaattagagtctcatattcactctcaactcgatcgaggcatgattgaacaagatggattgcacgcaggttctccggccgcttgggtggagaggctattcggctatgactgggcacaacagacaatcggctgctctgatgccgccgtgttccggctgtcagcgcaggggcgcccggttctttttgtcaagaccgacctgtccggtgccctgaatgaactccaagacgaggcagcgcggctatcgtggctggccacgacgggcgttccttgcgcagctgtgctcgacgttgtcactgaagcgggaagggactggctgctattgggcgaagtgccggggcaggatctcctgtcatctcaccttgctcctgccgagaaagtatccatcatggctgatgcaatgcggcggctgcatacgcttgatccggctacctgcccattcgaccaccaagcgaaacatcgcatcgagcgagcacgtactcggatggaagccggtcttgtcgatcaggatgatctggacgaagagcatcaggggctcgcgccagccgaactgttcgccaggctcaaggcgcggatgcccgacggcgaggatctcgtcgtgacccacggcgatgcctgcttgccgaatatcatggtggaaaatggccgcttttctggattcatcgactgtggccggctgggtgtggcggaccgctatcaggacatagcgttggctacccgtgatattgctgaagagcttggcggcgaatgggctgaccgcttcctcgtgctttacggtatcgccgctcccgattcgcagcgcatcgccttctatcgccttcttgacgagttcttctgagcgggactctggggttcggactctagctagagtcaagcagatcgttcaaacatttggcaataaagtttcttaagattgaatcctgttgccggtcttgcgatgattatcatataatttctgttgaattacgttaagcatgtaataattaacatgtaatgcatgacgttatttatgagatgggtttttatgattagagtcccgcaattatacatttaatacgcgatagaaaacaaaatatagcgcgcaaactaggataaattatcgcgcgcggtgtcatctatgttactagatcgaccggttggtacgaattcctgcaggtcaacatggtggagcacgacacacttgtctactccaaaaatatcaaagatacagtctcagaagaccaaagggcaattgagacttttcaacaaagggaaatatcgggaaacctcctcggattccattgcccagctatctgtcacttcatcaaaaggacagtagaaaaggaaggtggcacctacaaatgccatcattgcgataaaggaaaggctatcgttcaagatgcctctgccgacagtggtcccaaagatggacccccacccacgaggagcatcgtggaaaaagaagacgttccaaccacgtcttcaaagcaagtggattgatgtgataacatggtggagcacgacactctcgtctactccaagaatatcaaagatacagtctcagaagaccaaagggctattgagacttttcaacaaagggtaatatcgggaaacctcctcggattccattgcccagctatctgtcacttcatcaaaaggacagtagaaaaggaaggtggcacctacaaatgccatcattgcgataaaggaaaggctatcgttcaagatgcctctgccgacagtggtcccaaagatggacccccacccacgaggagcatcgtggaaaaagaagacgttccaaccacgtcttcaaagcaagtggattgatgtgatatctccactgacgtaagggatgacgcacaatcccactatccttcgcaagaccttcctctatataaggaagttcatttcatttggagaggacctcgagaattctcaacacaacatatacaaaacaaacgaatctcaagcaatcaagcattctacttctattgcagcaatttaaatcatttcttttaaagcaaaagcaattttctgaaaattttcaccatttacgaacgatagttaattaaccatgagcaagctcgagaagtttaccaactgctacagcctctctaagaccctcaggttcaaggctatccctgtgggaaagacccaagagaatatcgacaacaagaggctcctcgtcgaggatgagaagagagctgaagattacaagggcgtgaagaagctcctcgacaggtactacctcagcttcatcaacgatgtgctccacagcatcaagctcaagaacctcaacaactacatcagcctcttccgtaagaaaaccaggaccgagaaagagaacaaagagcttgagaacctcgagatcaacctccgtaaagagatcgccaaggctttcaagggaaacgagggatacaagagcctcttcaagaaggatattatcgagacaatcctgcctgagttcctggacgataaggatgagatcgctctcgtgaacagcttcaacggattcactactgccttcaccggattcttcagaaacagggaaaacatgttcagcgaagaggccaagagcacctctatcgctttcagatgcatcaacgagaacctcacgcgttacatcagcaacatggacatcttcgagaaggtggacgccatcttcgataagcacgaggtgcaagaaatcaaagagaagatcctcaacagcgactacgacgtcgaggacttttttgaaggggagttcttcaacttcgttctcacccaagagggcatcgacgtgtacaacgctattatcggaggattcgtgaccgagtctggggagaagattaagggactcaacgagtacatcaacctgtacaaccagaaaacgaagcagaagctcccgaagttcaagccgctctacaagcaggttctctctgatcgtgagagcctctcattttacggtgagggttacacctctgacgaggaagtgcttgaggttttccgtaacaccctcaacaagaacagcgagatcttctcgtccatcaagaagttggagaagcttttcaagaacttcgacgagtacagcagcgctgggatcttcgttaagaacggacctgctatcagcaccatcagcaaggatattttcggcgagtggaacgtgatcagggacaagtggaatgctgagtacgatgacatccacctcaagaagaaggctgtcgtcactgagaagtacgaggatgacaggcgtaagtcgttcaagaagatcggctctttcagcctcgagcagcttcaagaatacgctgatgctgatctcagcgtggtcgagaagctcaaagagatcatcatccagaaggtcgacgagatctacaaggtgtacgggtcctctgagaagttgttcgatgctgatttcgtcctcgagaagagtctgaagaagaacgacgctgtcgtcgcgatcatgaaggatttgctcgacagcgtgaagtccttcgagaactatatcaaggccttcttcggagagggcaaagagactaatagggacgagtctttctacggggatttcgtgctcgcttacgatatcctcctcaaggtggaccatatctacgacgccatcagaaactacgtgacccagaagccttacagcaaggacaagttcaagttgtactttcagaacccgcagttcatgggcggatgggacaaagacaaagagacagattacagggccaccatcctcaggtacgggtctaagtactacctggccatcatggacaagaaatacgccaagtgcctccaaaagatcgacaaggatgacgtgaacgggaactatgagaagatcaactacaagctccttccgggaccgaacaagatgcttcctaaggtgttcttcagcaagaaatggatggcctactacaacccgtctgaggacatccagaaaatctacaagaacgggaccttcaagaaaggcgacatgttcaacctcaacgactgccacaagctcatcgatttcttcaaggacagcatctcgcgttacccgaagtggtctaacgcttacgactttaacttcagcgagacagaaaagtacaaggatatcgccgggttctaccgtgaggttgaggaacagggttacaaggttagcttcgagagcgcctccaagaaagaggttgacaagttggtcgaagagggcaagctctacatgttccagatctataacaaggacttctccgacaagagccacggaactcctaacctccatacgatgtacttcaagctgcttttcgacgagaacaaccacgggcagatcagactttctggtggtgctgaactcttcatgcgtagggcctcactcaagaaagaagagttggttgttcacccggccaactctccaatcgctaacaagaatcctgacaacccgaaaaagaccaccacgctgtcttacgacgtctacaaggacaaaaggttcagcgaggaccagtacgagcttcatatcccgatcgctatcaacaagtgcccgaagaacatcttcaagatcaataccgaggtgagggtgctgctcaagcacgatgataacccttacgtgatcggaatcgatcgtggtgagagaaacctcctctacatcgttgtggtggacggaaagggaaacatcgtcgagcagtacagcctgaacgagattatcaacaatttcaacggcatcaggatcaagaccgactaccactcactcctcgataagaaagaaaaagagcgtttcgaggccaggcagaactggacttctatcgaaaacatcaaagagttgaaggccggctacatctctcaggtggtgcataagatctgcgagctggtggaaaagtacgatgctgtgatcgctcttgaggacctcaactctgggttcaagaacagtagagtgaaggttgagaagcaggtctaccaaaagttcgagaagatgctcatcgacaagctcaactacatggtggacaaaaagagcaacccttgcgctaccggtggtgctcttaagggataccagatcacgaacaagttcgagtccttcaagagcatgagcacccagaacggcttcatcttctatatccctgcttggctcaccagcaagatcgatccttctactggtttcgtgaacctgctcaagaccaagtacacctcgatcgccgacagcaagaagttcatctcgtctttcgacaggatcatgtacgtgccggaagaggatcttttcgagttcgctctcgactataagaacttcagcaggaccgacgccgactacattaagaagtggaagctctactcctacgggaaccgtatcaggatcttccgaaatccgaagaaaaacaacgtgttcgactgggaagaagtgtgcctcacctctgcctacaaagaactgttcaacaagtacggcatcaactaccagcagggtgatatcagggctcttttgtgcgagcagagcgacaaggcattctacagctcattcatggccctcatgtctctcatgctccagatgaggaactctatcaccggaaggaccgatgtggacttccttatctctccggtcaagaactctgacgggatcttctacgacagccgtaactatgaggctcaagagaacgctatcctgccgaagaatgctgatgcaaacggggcttacaacattgcgagaaaggttctctgggctatcgggcagtttaagaaagcggaagatgagaagctggacaaggtgaagatcgccatctccaacaaagagtggcttgagtacgctcagacctccgttaagcacaagaggcctgctgctactaagaaagctggtcaggctaagaagaagaaatgaggatcccgggcccgtcgactgcagaggcctgcatgcatcgaatttccccgatcgttcaaacatttggcaataaagtttcttaagattgaatcctgttgccggtcttgcgatgattatcatataatttctgttgaattacgttaagcatgtaataattaacatgtaatgcatgacgttatttatgagatgggtttttatgattagagtcccgcaattatacatttaatacgcgatagaaaacaaaatatagcgcgcaaactaggataaattatcgcgcgcggtgtcatctatgttactagatcgggaagcttcggaagacatcttgtgagaccgaggtctcaggtagtctagagtcgacggtatcgactttttttttgtttatcagcttacattttcttgaaccgtagctttcgttttcttctttttaactttccattcggagtttttgtatcttgtttcatagtttgtcccaggattagaatgattaggcatcgaaccttcaagaatttgattgaataaaacatcttcattcttaagatatgaagataatcttcaaaaggcccctgggaatctgaaagaagagaagcaggcccatttatatgggaaagaacaatagtatttcttatataggcccatttaagttgaaaacaatcttcaaaagtcccacatcgcttagataagaaaacgaagctgagtttatatacagctagagtcgaagtagtgattgaaattactgatgagtccgtgaggacgaaacgagtaagctcgtctaatttctactaagtgtagatggagacgttaatggatacgtctcggccggcatggtcccagcctcctcgctggcgccggctgggcaacatgcttcggcatggcgaatgggacttttttttctagaggtaatatggtttaaactatcagtgtttgacaggatatattggcgggtaaacctaagagaaaagagcgtttattagaataacggatatttaaaagggcgtgaaaaggtttatccgttcgtccatttgtatgtgcatgccaaccacagggttcccctcgggatcaaagtactttgatccaacccctccgctgctatagtgcagtcggcttctgacgttcagtgcagccgtcttctgaaaacgacatgtcgcacaagtcctaagttacgcgacaggctgccgccctgcccttttcctggcgttttcttgtcgcgtgttttagtcgcataaagtagaatacttgcgactagaaccggagacattacgccatgaacaagagcgccgccgctggcctgctgggctatgcccgcgtcagcaccgacgaccaggacttgaccaaccaacgggccgaactgcacgcggccggctgcaccaagctgttttccgagaagatcaccggcaccaggcgcgaccgcccggagctggccaggatgcttgaccacctacgccctggcgacgttgtgacagtgaccaggctagaccgcctggcccgcagcacccgcgacctactggacattgccgagcgcatccaggaggccggcgcgggcctgcgtagcctggcagagccgtgggccgacaccaccacgccggccggccgcatggtgttgaccgtgttcgccggcattgccgagttcgagcgttccctaatcatcgaccgcacccggagcgggcgcgaggccgccaaggcccgaggcgtgaagtttggcccccgccctaccctcaccccggcacagatcgcgcacgcccgcgagctgatcgaccaggaaggccgcaccgtgaaagaggcggctgcactgcttggcgtgcatcgctcgaccctgtaccgcgcacttgagcgcagcgaggaagtgacgcccaccgaggccaggcggcgcggtgccttccgtgaggacgcattgaccgaggccgacgccctggcggccgccgagaatgaacgccaagaggaacaagcatgaaaccgcaccaggacggccaggacgaaccgtttttcattaccgaagagatcgaggcggagatgatcgcggccgggtacgtgttcgagccgcccgcgcaagtctcaaccgtgcggctgcatgaaatcctggccggtttgtctgatgccaagctggcggcctggccggccagcttggccgctgaagaaaccgagcgccgccgtctaaaaaggtgatgtgtatttgagtaaaacagcttgcgtcatgcggtcgctgcgtatatgatgcgatgagtaaataaacaaatacgcaaggggaacgcatgaaggttatcgctgtacttaaccagaaaggcgggtcaggcaagacgaccatcgcaacccatctagcccgcgccctgcaactcgccggggccgatgttctgttagtcgattccgatccccagggcagtgcccgcgattgggcggccgtgcgggaagatcaaccgctaaccgttgtcggcatcgaccgcccgacgattgaccgcgacgtgaaggccatcggccggcgcgacttcgtagtgatcgacggagcgccccaggcggcggacttggctgtgtccgcgatcaaggcagccgacttcgtgctgattccggtgcagccaagcccttacgacatatgggccaccgccgacctggtggagctggttaagcagcgcattgaggtcacggatggaaggctacaagcggcctttgtcgtgtcgcgggcgatcaaaggcacgcgcatcggcggtgaggttgccgaggcgctggccgggtacgagctgcccattcttgagtcccgtatcacgcagcgcgtgagctacccaggcactgccgccgccggcacaaccgttcttgaatcagaacccgagggcgacgctgcccgcgaggtccaggcgctggccgctgaaattaaatcaaaactcatttgagttaatgaggtaaagagaaaatgagcaaaagcacaaacacgctaagtgccggccgtccgagcgcacgcagcagcaaggctgcaacgttggccagcctggcagacacgccagccatgaagcgggtcaactttcagttgccggcggaggatcacaccaagctgaagatgtacgcggtacgccaaggcaagaccattaccgagctgctatctgaatacatcgcgcagctaccagagtaaatgagcaaatgaataaatgagtagatgaattttagcggctaaaggaggcggcatggaaaatcaagaacaaccaggcaccgacgccgtggaatgccccatgtgtggaggaacgggcggttggccaggcgtaagcggctgggttgtctgccggccctgcaatggcactggaacccccaagcccgaggaatcggcgtgacggtcgcaaaccatccggcccggtacaaatcggcgcggcgctgggtgatgacctggtggagaagttgaaggccgcgcaggccgcccagcggcaacgcatcgaggcagaagcacgccccggtgaatcgtggcaagcggccgctgatcgaatccgcaaagaatcccggcaaccgccggcagccggtgcgccgtcgattaggaagccgcccaagggcgacgagcaaccagattttttcgttccgatgctctatgacgtgggcacccgcgatagtcgcagcatcatggacgtggccgttttccgtctgtcgaagcgtgaccgacgagctggcgaggtgatccgctacgagcttccagacgggcacgtagaggtttccgcagggccggccggcatggccagtgtgtgggattacgacctggtactgatggcggtttcccatctaaccgaatccatgaaccgataccgggaagggaagggagacaagcccggccgcgtgttccgtccacacgttgcggacgtactcaagttctgccggcgagccgatggcggaaagcagaaagacgacctggtagaaacctgcattcggttaaacaccacgcacgttgccatgcagcgtacgaagaaggccaagaacggccgcctggtgacggtatccgagggtgaagccttgattagccgctacaagatcgtaaagagcgaaaccgggcggccggagtacatcgagatcgagctagctgattggatgtaccgcgagatcacagaaggcaagaacccggacgtgctgacggttcaccccgattactttttgatcgatcccggcatcggccgttttctctaccgcctggcacgccgcgccgcaggcaaggcagaagccagatggttgttcaagacgatctacgaacgcagtggcagcgccggagagttcaagaagttctgtttcaccgtgcgcaagctgatcgggtcaaatgacctgccggagtacgatttgaaggaggaggcggggcaggctggcccgatcctagtcatgcgctaccgcaacctgatcgagggcgaagcatccgccggttcctaatgtacggagcagatgctagggcaaattgccctagcaggggaaaaaggtcgaaaaggtcactttcctgtggatagcacgtacattgggaacccaaagccgtacattgggaaccggaacccgtacattgggaacccaaagccgtacattgggaaccggtcacacatgtaagtgactgatataaaagagaaaaaaggcgatttttccgcctaaaactctttaaaacttattaaaactcttaaaacccgcctggcctgtgcataactgtctggccagcgcacagccgaagagctgcaaaaagcgcctacccttcggtcgctgcgctccctacgccccgccgcttcgcgtcggcctatcgcggccgctggccgctcaaaaatggctggcctacggccaggcaatctaccagggcgcggacaagccgcgccgtcgccactcgaccgccggcgcccacatcaaggcaccctgcctcgcgcgtttcggtgatgacggtgaaaacctctgacacatgcagctcccg

SEQ ID NO: 21 - DNA, 28 bp, Artificial Sequence
  DnaJ domain-containing protein Oligo for guide Forward
agatggcagagatgtaaacatcaaatgg

SEQ ID NO: 22 - DNA, 28 bp, Artificial Sequence
  DnaJ domain-containing protein Oligo for guide Reversed
cggcccatttgatgtttacatctctgcc

SEQ ID NO: 23 - DNA, 28 bp, Artificial Sequence
  XRI1-like protein Oligo for guide Forward
agattagttatggagagcactccaccag

SEQ ID NO: 24 - DNA, 28 bp, Artificial Sequence
  XRI1-like protein Oligo for guide Reversed
cggcctggtggagtgctctccataacta

SEQ ID NO: 25 - DNA, 28 bp, Artificial Sequence
  XRI1-like protein Oligo for guide Forward
agatgccagataaccaagtgtgatagcg

SEQ ID NO: 26 - DNA, 28 bp, Artificial Sequence
  XRI1-like protein Oligo for guide Reversed
cggccgctatcacacttggttatctggc

SEQ ID NO: 27 - DNA, 28 bp, Artificial Sequence
  DnaA initiator-associating diaA protein Oligo for guide Forward
agatgccttactacctggtcctgctggg

SEQ ID NO: 28 - DNA, 28 bp, Artificial Sequence
  DnaA initiator-associating diaA protein Oligo for guide Reversed
cggccccagcaggaccaggtagtaaggc

SEQ ID NO: 29 - DNA, 28 bp, Artificial Sequence
  DnaA initiator-associating diaA protein Oligo for guide Forward
agatgttgctagactcatgggtttggag

SEQ ID NO: 30 - DNA, 28 bp, Artificial Sequence
  DnaA initiator-associating diaA protein Oligo for guide Reversed
cggcctccaaacccatgagtctagcaac

SEQ ID NO: 31 - DNA, 28 bp, Artificial Sequence
  TAF-2 protein Oligo for guide Forward
agatacatggcagtagctggtcgactcg

SEQ ID NO: 32 - DNA, 28 bp, Artificial Sequence
  TAF-2 protein Oligo for guide Reversed
cggccgagtcgaccagctactgccatgt

SEQ ID NO: 33 - DNA, 28 bp, Artificial Sequence
  TAF-2 protein Oligo for guide Forward
agatacccaaagagtcgaccagctactg

SEQ ID NO: 34 - DNA, 28 bp, Artificial Sequence
  TAF-2 protein Oligo for guide Reversed
cggccagtagctggtcgactctttgggt

SEQ ID NO: 35 - DNA, 28 bp, Artificial Sequence
  Phosphoethanolamine N-methyltransferase protein Oligo for guide Forward
agatcctgaatcagtggacttgatattg

SEQ ID NO: 36 - DNA, 28 bp, Artificial Sequence
  Phosphoethanolamine N-methyltransferase protein Oligo for guide Reversed
cggccaatatcaagtccactgattcagg

SEQ ID NO: 37 - DNA, 28 bp, Artificial Sequence
  Phosphoethanolamine N-methyltransferase protein Oligo for guide Forward
agatactggggacttagccgagaaggcg

SEQ ID NO: 38 - DNA, 28 bp, Artificial Sequence
  Phosphoethanolamine N-methyltransferase protein Oligo for guide Reversed
cggccgccttctcggctaagtccccagt

SEQ ID NO: 39 - DNA, 28 bp, Artificial Sequence
  eEF1B protein Oligo for guide Forward
agatacctcacccaatatcttgacgaag

SEQ ID NO: 40 - DNA, 28 bp, Artificial Sequence
  eEF1B protein Oligo for guide Reversed
cggccttcgtcaagatattgggtgaggt

SEQ ID NO: 41 - DNA, 28 bp, Artificial Sequence
  eEF1B protein Oligo for guide Forward
agatatgcagctactgcaccttcctcag

SEQ ID NO: 42 - DNA, 28 bp, Artificial Sequence
  eEF1B protein Oligo for guide Reversed
cggcctgaggaaggtgcagtagctgcat

SEQ ID NO: 43 - DNA, 28 bp, Artificial Sequence
  Tetratricopeptide repeat (TPR)-like superfamily protein Oligo for guide Forward
agatccactagtccccgacggcccaaag

SEQ ID NO: 44 - DNA, 28 bp, Artificial Sequence
  Tetratricopeptide repeat (TPR)-like superfamily protein Oligo for guide Reversed
cggcctttgggccgtcggggactagtgg

SEQ ID NO: 45 - DNA, 28 bp, Artificial Sequence
  Adenylyl cyclase-associated protein Oligo for guide Forward
agatggtccaggattgagaaaggtgacg

SEQ ID NO: 46 - DNA, 28 bp, Artificial Sequence
  Adenylyl cyclase-associated protein Oligo for guide Reversed
cggccgtcacctttctcaatcctggacc

SEQ ID NO: 47 - DNA, 28 bp, Artificial Sequence
  Adenylyl cyclase-associated protein Oligo for guide Forward
agatgtggtgcagatacagctactttcg

SEQ ID NO: 48 - DNA, 28 bp, Artificial Sequence
  Adenylyl cyclase-associated protein Oligo for guide Reversed
cggccgaaagtagctgtatctgcaccac

SEQ ID NO: 49 - DNA, 21 bp, Artificial Sequence
  U6pro-F Oligo Forward
aggcatcgaaccttcaagaat

SEQ ID NO: 50 - DNA, 2889 bp, Artificial Sequence
  DnaA initiator-associating diaA CDS
atgaatgatagtttagccataacagcatcatcattggccattactgagaaaaagcctcaaaggcctgggggttgtgtgggtattttctttcaactctttgattggaaccgtagatttgccaagaagaagttgtttccaaagaaactgctttcaccagctcgcttgaaacaagcttcaaagaagtttggaggggatgaaaagcagccaaagcatcgtttgattgctaatgagaatagtgggggttttccaattgcaaagagcaacggaatgagcaatactcgttgtgaaagcaagcgcgaaatgaaagcaccaagtttggttgctagactcatgggtttggaatcaatgccagcaggaccaggtagtaaggccaaaaaggcttcagcttctgaaactgggagctatgtggcggagaaacttgatgctcggcctggcggatctgataaagaagatatggattgtgagaaggctgaaataaagcgtgaattgaggccccaaaagcttcagaagataggggtgagtgagagacgtccagtcagcagatttagtgctgaagcattgcagttgaggactgtattgtcaaggccaaggaaacatcagcctaaattgacttctccagtaaaaagtcctagaaacgtctctggtagaaatgcatctaggttgattggggctgcaactaggattttggaaccgggtttgcaaaagagtagggcgaaatgtgctcttacttatcctaaatatttttctcctttggaagataaagcagatttagcactgcatcatttggaagtccctaatccttgtgtggattcaaagacttcggaagtgagagcatctgtgccttcatgtaaaaattgtggttatatgcttcatagtaagaatggtacaccaaatggggaagaacacccatcgtctgtctcgtcacctgtctctagttactctcaaccttcttgtcaaggtccaggaagaaatatgctaaggttgcccattatcaacagcagagatcaattagagagagtttttgagggttcgtcttcagacgccaatgctgaaatagatgatgtatcatactgtgcagagctcatattgggcaagcgacctattagcagaagtcgaatagcgatgcatggcgcctgccaagggagcaatgtgaaaaaggatgcatcatctgtcactcatgtgcttaaccagaagcaaaatcaaacatctcagaatagagagaggggatttatgaagtctaagcaaagtagtttgcagagcaacagagttttagcagctgcagaatctacgattaataccaaaagttttgttgcacagaatagaaggttaggtgcatctacccgattgagaatgccagccacagccgatggctgcaagtttgaaactgaaagaaaaccttattcaaggagaagtgattccctctctccggtgcggaagaagagattgatgaatgtctccagacaaggtgaaagttctagttttgtgaatgcgaatttgggaagagaatcaagcccttattctgacaaaacaagtagaaaagatgttttcccaatttcttccgttaatagtcactccactaaaccgaagttgccatgtttgcgagagagtggtgcaaccaataatagttctgagggaagtaatgttgtttcgtttacttttagatctgcaatgaagcagaaagctggcattcatgcagaagtcacaaaaaggaagtctcaaaatagctcaagttttgatgctactccagggagatccttctttactggaaatgatgaaacagcatgcttgcagaaatcctttcctttgaaaggagacattttaggagcacttttggagcaaaagctaaaggaattgactagtgaagaagagttcgcagaaggagatgctgcacctagaaaaagcactgcaacgatccttcaggagctaataactgctttgaatgatgagacccaatttcatctggatagtttgccttctaaacctaacagaaaagaagatttgtatgatgatcgtgaagtgtcttcaagaaatacttccatgaatttccaggccataccagattcagcaaccgatttagttgggaattcacttgataatgatcaccttagtccaggatgtgttcttgaagctaccttttcaactgacagctacctctccagcagtcccaatagtagctcaaaggacaaagtgcttgccgaatctgtggactctatttatgacgaaccactctttccagaacctgatagagatctttcggattgtgcgacctcattattcaccaggaggagttgcagagcactgatcacagaccatgttaacaacatttctggagtgctaagcaagattaatcagttaaaaggaagcaaactcggttatgcaaatgaggtcattttgaatactgaactcatacttggaacctcacctgaacaacaggctttacctgtagacgatgggttatcagtgagccattttctcctcaatgaacttgaaatgctatcaagtcttctatggatgacttttggtcagttgcttggctgtaacgaccccaaacagatgaatcagcttaaaggatttgcctttgattgtctattagagtatctagactcaaaatttggtcgatactctgattctggtttcagaatctggtctaaactaccatcaagcatgactaaagagattctgattgctgatattattgaagaggtcaaagagtggacggaatttgttgggttgatccccgacgagctaatagaatgggatatgagccattctttgggtaaatggacggattttgagattgaagaatttgaatgtggcactgaagttgataggcatattctccaagtattagtagatgaagttgttttggacctctacagttctagttaa

SEQ ID NO: 51 - DNA, 1668 bp, Artificial Sequence
  TAF-2 CDS
atggctggtgagaagattatagaaaaacctgaagctgttgctccgggactgaaatctgatccctctaacaaactgattgagaaggatttggtttcaaaaaaagatggaaaagctgctgactcggtggcttctttgggagctgtgaccagcatcaagtgtgaaaatgatcaaccacctgctgcagagcaaggatataatgggacttataatcagttagatgagcaggcttactttaatgcgggtgttcaatcagacaatggttcccttctctactatatgcctggctataatccttacagtgctggatttgtgggaggcgatgggaagcagccctatccttcgtccggatatctccagcaacctgtctcatatggttcagattccatgccatgttatacatggggctcgccatactgtgctgatatcaccaatagtgctgctccaaaatccgggaacgttaaatcaacttttggacgaaatggttcagtcaagtcgaatggttttaattccacaaaaacaaatagttctttctcaagcaaaaactcgaccgtactctttaacccaaagagtcgaccagctactgccatgtcaaatcctccaaagtctttccatcaagctcagccttttaatccagtgaacaagtttcagtccgatgtccagtctggaggcctgatgaaggggtttcatctggttggggactacccatcatacacgagtcagaatcaaggttttttcatgccttatgatcccatcaactgtcaaacaaacagtagaatgtggaatggaaactacagagctaaaccacggggaaatttcaccagaaatggtgtgtttgaggcaactaatgagttacctcgtggtccccgtgccaacggtagaagtgtcccttcaaaaccatctgctgaggaggatcagcttgtgccagctgttcagagggagaagtataacaaggaggattttaagactcagtatgacaatgcaaaattttacattatcaagtcatacagtgaagatgatatccacaagtgtgtcaaatatgatgtgtggtcaagtactccaaatggaaacaagaaattggacactgcctttgttgaatctgaggctaaagcaagtggaactggttcaagctgtccagtgttcctcttcttttctgtaaatggaagtggacagtttttaggtgtagctgagatggttgggcaggttgacttcaacagaaacatggacttttggcagcttgataagtggagtgggttcttcccactgaagtggcacatagttaaagatgtaccaaatacacagttcaggcacatcatccttgaaaacaatgataatagacctgtaacctatagcagagatacacaggagattggattgaaggaaggtttggaaatgcttaacatacttaagaattactcagagaagacatctatattggatgatttcaatttctatgagaagcgtgagaaagtgctcaaggctaaaaggagttcaaaaccagttattcaagctgatgcatacgagaaagctgattctcttaagcaattcaaaggaggagacaaggtactcgaggaggagctgaagaccaactctactgatccaactgcacctttggtttctctcaccaaaaacctatcgattaattcaaggccattcaaaagtagtgtctga

SEQ ID NO: 52 - DNA, 1416 bp, Artificial Sequence
  Adenylyl cyclase-associated CDS
atggatgagaagttgatacagcgattggagtccgccgtgtcaaggctggaggcgctttcagtcggcggcggtgtttcacttggagatggagaagctgcggcggctttagatccatccattattgcatttgatgatctgaggtcacggttcgtcggtagagtttgcactgctgcagagaagattggtggacaggttttggatgtcactaagattgttgaggaggcttttgaagctcagagagaacttcttatcaaaatcaaggaaactcagaaacctagcatgtctggtttggctgaatttcttaagcctctgaatgatgtgatagtgaaaggtactaaaatgacagaaggacggcgatctgatttgttcaaccacctgaaggctgctgttgatagtctaacagccctggcatggatcgcatacactggaaaagattgtggtatgagtatgcctattgcacatgtggaagaaagctggcagatggcagagttttacaataacaaggtccttgtggagttcagaaacaaagacccagatcatgttgaatgggcaaaagctttgaaagagatttatctccctggcttgcgggattacgttaagagtcactacccattgggccccgcgtggagtgctacagggaaagtagctgtatctgcaccaccaaaagctcccgcaccaagtcgtcccatgcctcctccactgccaccagcttctttattcagctcggaatctccccaggcttcatcatcacgccccaagaaagggatgtcagctgtttttgatgaaattaattcggggaagccagtcaccggtggattgagaaaggtgacagatgatatgaagacaaagaatcgtgcagatagaaccggtgtcattagtgcaggagaaaaggaacgtcgcgttagctcaccatctttctccaaagctggacctccaaaactggagcttcagatgggtcgtaaatgggtggttgagaatcaaataggaagaaagaatctagtcattgatgattgtgatgcaaagcaatctgtctatatttttgggtgcaaagattcagtcctgcagatccaagggaaagtcaacaacataacaattgataagtgtactaaaatgggagttgtattctcggatgttgtggcagcttgtgaggttgtcaactgtaatggtgtggaggttcaatgtcagggttcagcaccgactatttcagttgataatacaactggatgccaattatacttgagcaaagattctttggggacttccattacaacagccaagtcaagtgaaattaatgttttggttcctggtgcaggggctgatagtgattggggggagcacgctttgccacagcagttttctcatgtatataagagtggccaatttgtgactacacccgtctcacattcaggaggttaa

SEQ ID NO: 53 - DNA, 1485 bp, Artificial Sequence
  Phosphoethanolamine N-methyltransferase CDS
atggctgccattgctccagaggtaggagaagagcgtgagattcaaaagagttattggatggagcaaactagtgaactcaatttggaggcaatgatgcgtgattctgcagcatctgatcttgacaaagaggataggcctgaggtgctttcactgctcccttcatatgaaggtaaatccgtgttggaattgggtgctggtattggccgtttcactggggacttagccgagaaggctggggagcttgtagcagtggactttattgaagaagtgactaagaagaatgaaagtatcaacgggcaccacaagaatgtcaagtttgtgtgtgctgatgtgacttcaccagatttgacggttttacctgaatcagtggacttgatattttctaactggctactgatgtatctttccaacgaagaggttcaggaccttgcggagagaatgatcaaatggttgaaagttggtggctatatattttttagagagacatgcttccatcaatcaggagaccacaagggaaagaacaacccaacccactatcgagagcctcgattttatacaaaggttttccaagaatgtactttaaaggatgatgctggaaaatcatatgaactttctcttattggttataagtgcattgaaacttatgtaaaaaacaaaaagaatcaaaatgagatttgctggatatggcagaaggttcattccgaggatgacaggggattccagcatttcttggacactgttcagtacaagtctaatggtatactgagatatgaacgtgtgttcggggcaggctttgtcagcacaggaggaattgacaccaccaaagaattcgttgccatgatggatcttcagcctggcgaaaaggtccttgacgttggctgtggcattggaggaggtgacttttacatggctgagaagtatgatgttcatgttgtaggcattgatctttcagttaacatgatcacattggcttttgaacgtgctattgggcgcaaatgcgcggttgaatttgaggttgctgattgcacggtgaaaacatatcctgaagaatcattcgatgtgatatacagccgggacactatcctgcacatccaggacaagcctgcattattcagatctttctataagtggctgaagcctggaggcagagtcctcataagcgattactgcaaaaaggcaggaccagcttccgaagactttgcagcgtatatcaaacaaagaggctacgatttacatgatgttgaagcatatggacagatgcttagagatgctggtttcaacgaagttattgctgatgatcgaactgagcagttcatgcaagttctccagaaagagttggatactgtggagaatgaaagagagttatttatccaagaattttctgaacaagactacaatgatatagttggaggttggaaggccaagctagttagaagttcatctggtgagcagagatggggtttgttctttgccaagaaaaattga

SEQ ID NO: 54 - DNA, 1527 bp, Artificial Sequence
  DnaJ domain-containing protein CDS
atggagtgtaataaagatgaagccttcagagcaaaaaaaattgcagagcggaagtttgaacagaaggattatgctggtgcaaagaaatttgccttgaaagctcaggttttgtatccagggcttgacgatttaacccagatgttaacaacatttgatgtttacatctctgccgaaaacaaagtaagtggggaagtggattggtatggggtacttggtgtgagcccgtcaagtgatgatgaaacggtaaagaaacagtacaggaagctagctcttgtcctccaccctgataaaaataaatctattggtgctgaaggtgcatttcaacttctctctgaggcctggagcttgttatctgataaatccaagaggttggcatataaccagagaaggagttcaaaaggtccccagcagaaacaacagaaagttccagtgccctcaggtggtccatcaactttctggaccatttgccaccgttgcaagatgcattacgagtatttgaagatatatctcaaccacactcttctttgccccaactgtcatgaatctactagtcagtggaaaagagaacggagattgaagggagtaaagaaagtaccagatcctgattttcacaatttcgatcaggataggagcgaaagttgttttgaagacaatgaagtctgggcttcatatgatgctgatgatggcatgccccgtttctatgctctgattaacaaagtcatctcaagggaaccatttaaagtgaggctcagttggcttaattcaaaaacgaacactgaatttggtccaatggagtgggtagcttcaggtttctataaaacttctggtgagtttaggattggcagatatgaaacgggtaagtcggtgaattccttctcccacaaggttcgatggtcaaagggccctcgtggaactgttctaatatatccccaaaagggggatgtttgggccctcttcagaaattggtctgctgactggaatcagaatacacctgatgatgttatacacaagtatgacatggtcctagttcttgatgattacaatgaggagcaaggaatttcagtagctcctctcatcaaagttgctggttttaagacagtctttcgtccagacttgaatccggagaagatgattagaataaccagagaagagatgtttcgtttctctcatcaggtcccaagccacttgcttacaggtgaagaaggtcaaaatgctccaaagggttgccaggagcttgatccagctgctactccattggagcttcttcagacagtaacagaaactaatgaggtgccagccatgcagaacgacaaggaggctaatggaggttcatcacagaaagttcaggaaacaaaaactagtgaggctgctgatcatactctcaaatctagggaaggcgggatggtagaaagtgaaggagagattagtcttggttcagaacagatggttgagaaggttactatggagcaaacacaggttaatcctgtaaagactgacaaggctactaagtttggaactgagacgtag

SEQ ID NO: 55 - DNA, 1242 bp, Artificial Sequence
  Elongation factor 1-gamma 1 (eEF1B) CDS
atggctctgattttgcattcaacagacaacaacaaaaatgcctcaaaggcactcattgcagctgagtacacaggtgttaaggttgatcttgcaaaggacttccagatgggtgtatccaacaagacacctgagtttcttgagatgaatcccattggaaaggttcctgtgcttcaaacacctgatggacctgtttttgagagcaatgccattgcgcgttatgttaccaaaacaaagcccaacaatcctctttttggctcttcattgattgaatatgctcaaattgaacaatggaatgatttttctgccactgaaattgatgcaaacattgcacgatggctgtacccacgccttggctatgctgtttacatctctcaagctgaggaaggtgcagtagctgcattaaagagagcgcttggtgctttgaacacccatcttgcatctaacacatacttggttggacattttatcacactggctgacatcatcatggtctgtaacttgagcattggttttaggatgatattgaccaagagctttaccaaggaatttccacatgtagagagatatttctggactgttgttaatcagcctaatttcgtcaagatattgggtgaggtgaaacaagctgaatctatccctgctgtgcaatccaagcctgcacaacctgaaaaactcaaggctaaggaggagccaaagaaggaggttaagaaggaagaaccaagtcctgtagaggaggaagcagcacccaagcctaaggcaaagaatcctcttgatttattgcctccaagtaagatgattctggatgattggaagaggctttactccaacaccaagactaacttccgtgaggttgctgttaaaggtttctgggacatgtatgaccccgaaggatattctctctggttttgtgattacaagtacaatgatgagaacacagtttcgtttgtaaccttgaacaaggttggtggttttctgcagaggatggagctggtacgcaagtatgcttttggtaagatgttgattgttggttctgaggccccattcaaggtgcagggcttgtggcttttccgtgggaaggaaattcccaagtttgttatggaggaagtgtatgacatggaactctatgaatggaaggaagtagacatcaatgatgaggcccagaaggagcgagttagccaaatgattgaagatcacgagccttttgagggacaggctttgttggacgccaagtgcttcaagtaa

SEQ ID NO: 56 - DNA, 5775 bp, Artificial Sequence
  Tetratricopeptide repeat (TPR)-like superfamily CDS
atggcacccaacaagaatggtcgtggcaaaacaaagggagacaagaagaagaaagaagagaaggttctcccagttgtaatggatataacgataaaccttccggaggagactcaagttattttaaagggaatatctacggatagaattatcgatgttcgtcgattattatctgtcaatacaacaacttgtaatgtcactaatttctcactgtctcatgagttaaggggtccacgtttaaaagaaacagtggacgtttccgcactgaagccctgcatcctgactcttatcgaagaggaatacgatgaagaaagcgcaacggcgcatgttagaaggctgttggacatcgtcgcttgtacaacgagttttgggccgtcggggactagtggtaaagagttgaaaactgactcttgcaagaatgcgcgaggtgtgcaggataacaagaatgctaagaaatccaacaaggttcgtgggaatgataagtcatcgtcgccgccacaaacgccaactccggtggcgcaacagctgggtaaagatgcgggatcggaagaagttgatggagagatgagcaatacttgccctaagattggaagcttctatgagttcttctcgctttctcatctcacgcctcctcttcagtgtaatgcgccctctctctctcacattgtgtctctcttctcgtgtttcttgttaaaattaagactcatcttgattcttgcagtcataagaagagcaacaagacaacaagatgatgaagttttgccagatgatcatcttttctctcttgaagtgaaactttgtaatggaaagctggttattgttgaagcttgcaagaaaggattttacaactttggaaagcaggggattctttgtcacaatcttgttgatttgttgagacaactcagtagagcatttgacaatgcatacgatgatctcatgaaagcattcttggagcgtaataagtttgggaatcttccatacggattcagagccaacacatggcttataccacctgtggcagcacagttgccagctatttttccacctctacctgtggaggatgatacctggggagcaaatggaggtggtctaggccgagatggaaaatttgattctttaccttttgccaatgaatttttgaatgttgcatccatggcttgtaagacaacagaggagaggcagatcagagacaggaaggcttttattcttcatagtttatttgttgatgtcgccattttacgagccatttcagctgtaaagcatgtcatggagaaagttaaaccagctcattgtgatttgaatggagaaatcatttataatgagacagttggggacttgagcatatttgttaccaaagattcttcaaatgctagctgcaaagtagataccaaaattgatggatttcaagcaactggaatagctatgaagaatctgatggaaagaaatttactgaaggggataactgctgatgaaaatactgctgcccatgatattgctactttaggtgttctgaatgtaagacattgtggttatattgcaactgtaaaagttcaaggaaaagaaaatgacaaagtgggcagcccactgcaaagcatggaacttgctgatcagcctgatggtggtgcaaatgccctcaatatcaacagtttacgcttgctccttcacaagaaagtggacaacaaggtaatgcattcaaaaccttcagaaactgaagagcctaattgctctcaggcatttgtaaggagaatactagaagagagtcttaccaaacttgaagaagagaaaatagaaggtgactctttcatcagatgggaacttggtgcatgctggatacagcacttacaagatcagaaaaaatcagaaaaggacaagaaaccctccgctgagaagaaaaaaaatgagatgaaggttgagggacttggaatacctcttaagtcccttaagaacagaaagaagagcacagatggaactaacatggaatcccagtcagaaagcttcaaatctgccgcagatggtgttggagggggatcagaaaaacctgtcctgcagtctggggagtctcagtttgagacagatacagatcaaaatcaggtcgtcctcaaggcattgttgtctgatgctggctttacaaggttgaaggagtcagagactggacttcaccttaagtctttggaagagctgattgatctgtcacagaagtactataatgaagttgccctgccaaagctggtggctgattttggctctttagaactctcaccagtagatggtcgaaccttaactgatttcatgcatacccgaggtctacgtatgcgttctcttggacaagtagttaaactttctgagaagttatcacatgtgcaatctctttgtatacacgagatgatagtccgagcttttaaacatattcttcaagcagctattgcatcagttgttgacattgaagatatagctgcgataattgctgctgccttgaatatgatgcttggggtacctgaaaatgatgattcaaatgagtacggtgttgattctttgatctggagatggctgaaattatttttgaagaagagatacgaatgggatgttggcagcctgaactacaaagatatgaggaaatttgctatcctccgtggtttatgccataaggtgggaattgaactggttccaagagattatgatatgagttcagcaagtccttttcagaaagtagacattgtcagcctagtaccagtgcataagcaagctgcttgctcttctgcagacggaagacagcttttggaatcatccaaaacagctctggataagggaaaacttgaagatgcggtcagctatgggactaaggctcttgccaagctggtcgcagtatgtggtccataccatcgaatgacagctggagcttatagccttcttgctgttgttctgtatcacaccggtgattttaatcaggccacaatctatcagcaaaaggccttggacataaatgaaagagagttgggccttgatcacccagacactatgaaaagttatggtgatcttgcagttttctattaccgacttcaacacacagagttggctctcaagtatgtaaaacgagctctttatttgttgcatctcacatgtggcccctcccatccaaatactgcggcgacatatataaatgtggctatgatggaggaagggctcggtaatgtgcatgttgctctcagatatctccataaagctttgaagtgtaaccaaaagttactcggtccagaccatattcagacagctgcaagttatcatgctatagcaattgccctctctttgatggaagcttatcctttgagcgttcagcatgagcaaacaaccttgcagatacttcgagcaaagcttggtccagatgatcttcgcacacaggatgctgctgcatggcttgagtattttgagtcgaaggcttttgaacagcaagaagctgctcgaaatggaactaagaagcctgatgcatcaatagccagcaagggtcatttgagtgtgtcagatttgctcgactacattaatccaagtccagatgccaaagggagagatgttggatcaaaaagaagaggttttgtctcaaaggctcttatttctcaggtgaagggaaaatctgatcaaaacaatgttgccataccaaactctgacacttttaaagatgttccaaaagaagagacagatgaaaagaaacaaattgtcgaagatcacactgatcccaagatgaatatggaacctgttgacactgtaattgaatcccatcacaatggagatggaggaattactgagaacaaacccatccaatctggaccattgttaaaggaaacttcaattgagaagtctatggtccgtgaagtcttatctgaaccttctgctgaagcagaagatggatggcagccagtgcagagaccaaggtcaggtggtttctatggacgaagacgaaggcagaggcgtcaaaccatcagcaaggttattggttaccagaaaaaggacccaatttctgatgttgatcatgctaaattgaagaataactatcaagctagtaaatattatgtcttaaagaaacggacatcaccaggaagctatgcagattattacttagcaaaaagtcaggcttctggtaccaaacttggtcgaagagtcataaaagctgtagcctaccgtgtgaagtctgtgtcatcttctgtcagagatgctgttcctgagatctccacaactggaggagatttgttaaatacttcatcagagcaggtccaagtttctgcaacaaaggaggttggatcactatcaaagagaagttcaatagtaaacctaggaaaatctccttcctataaggaagtagcacttgccccgccaggtaccatttctatgttgcaggagagagtttctgaagatgaaattcctgataacccagacgttatgaaacttgaaaaggagagcaatggagcagaagaaaattccaaaataatgggaagagatgcagaatccatggagaaagagaacattcaggatctagttgcaaattcttctgatcatgtaaaaagtgaaacagtagatactgacagtaaagaagaaattcaaatgagtgatctcaaaggtggtgaaatttcagatctgatatctgcaaatgcatctattcaacccggccatgttgatgttagtccaatggaacagggtagtgtcaagactcataatgtccctacttctgacaattctcccaaagcggatccctgtgaaaaggactcatcaagcaatttaaatcctggcgttatctcaaatatgaccttgcaagatatggatcatctgaaggtaaaatctgcgtcatctcatgcaagtgatgccagtcgagaattgtccagaaagctatctgcatcagcagcaccattcagcccttccccagctgttccccgcggtaccccattacctatgaacattaatctcccttctcctcctggaacacgaccaccgattggtccttggtcagtgaccatgtctcttcatcaaggaccaccgaccatcttgcctagtccaatgtgctcctcccctcatcacctgtacccttcacctccacacaccccaaacatgatgcacccattgcgctttatctaccctccgtattctcaaccccagacgttacctccaaatacattccccatgagtagcagcactttccatccgaatcattatgcttggcaatgcaatatagctcctaatgcatcagagtatgttcctgccacagtttggcctggctgccacccagtcgagttttctatctcaccacctgtgattgagcctataactgactcaatttcctctgctaaggagatatctgataatcctgaaaatattactttgacaacaagcttactagttgatctcaacaccggggatgaagtcaaggaagatgtaaatcttccagcatcagaaacagtggagaacatagctgcagttgtaccagaaaaagagagagcaagcaacactccagattcacattttgttacctcgtctagtgatcaatcaaaagagggcagtggatcaaatcatgtgcaaagaaatcttacggagacggataatgagaagaccttcaacattttggtacggggccggaggaatcgcaaacaaactctaagaatgcctataagtttgctcaagagaccatattcttctcagcccttcaaagctgtatatagcagggtaataagggagactgaggttcccagctctaccagctttgatccacatgaacatggcataacgactgctacttga

SEQ ID NO: 57 - DNA, 753 bp, Artificial Sequence
  XRI1-like CDS
atgggtgaccttcactcaattgcttacaatagcttctcttccctaggttgtgacttccatggcctagaagttctcaacaatgatatgtctccatttatggagagcactccaccatttttgtcaaattttgattgtgagttgtcaagtggatatctacaagatgctttattcaaattcaactcaaaaagaaggcgtttatttttgtttaatgatgatgatgacaaggagaattatcaaaataaagattcaattaagaatttgtggagctccacaattgaccaacaattttctgaggattatgattcttttagccagataaccaagtgtgatagcttttctggggatccaatgagcaaaatgagtgaagaatattccaaaagaacagaggaggaagcaatctcagaaaattattattattcttctaattcttcaccaacatcatcatctcatcataataaacaacctctacaatatggaggaggtgataaaaagagaagaatgtgtggaaaaattgtgtatccatttgggctagtgaagcccggagggcaagaaggagacgtgacattaaatgacattaacgagaggattctaatgaggccgacccggcccgtaaggcatccggttggggactttgcatgtcgttcgaccgtatgccctgctggaccaggattatccggcaagacggtggttgcactcaccaaaattcatactcaagggagggggacaatcacaattataaggactcgagggtga

SEQ ID NO: 58 - DNA, 2910 bp, Artificial Sequence
  DnaA initiator-associating dia A CDS
atgaatgttagttcagctagagaaatgaatgatagtttagccataacagcatcatcattggccattactgagaaaaaacctcaaaggcctggtggttgtgtgggcattttctttcagctctttgattggaaccgtagatttgccaagaagaagttgtttccaaagaaactgctttcaccagatcgcttgaaacaagcttcaaaaaagtttggaggggatgagaagcagccaaagattcgtttgattgctaatgagaacagtgggggttttccaaatgtaaagaacaatggaatgaccaatacatgttgtgaaagcaagcgcaaaatgaaagctccaagtttggttgctaggctcatgggtttggaatcgatgccagcagcatcaggcagtaagcccaaaaaggcttcaggttctgaaattgggagcaatgtggcagagaaactcggtggtcaacctggcggatctgataaagaagatatggatttcgagaaggccgaaataaagcgtgaattgaggcctcaaaagcttcagaagatagggcttagcgagagacgttcagtttgcagatttagtgctgaagcattgcagttgaggactgtattgtcaaggccaaggaaacatcagcctaaattggtttctccagtaaaaagtcctagaaatgtctctggtagaaatgcatctaggttgattggcgctgcaactaggattttagaaccgggtttgcaaaagagtagagtgaaatgtgctctcacttatcctactagatatttttcccctttggaagataaagcagatttagcacctcatcatttggaaggccccaatccttgtgtggattcaaaaactttgaaaggaacatctgtgccttcatgtaaaaattgtggttattttcttcatagtaagaacggtataccaaatgtggaagaacactcatcgtctgtctcgtcacctatctctagttactctggacctccttgtcacggtccaggaagaaatattccaaagttgcccattttcagtagcagggatcaactagagagagtttctgagggttcgtcctcagacgccactgctgaaatagatgatgtatcatactgtgcagaactcatattgggcaaaagatctattagcagaagtcgaatggagatgcatggcacccgccaagggaacaatgtgaagaaggatgcatcacctgtcactcatgtgcttaatcagaaacaaaatcaaacatctcagaatagagagaggggccttatgaagtctaagccaagtagtttgcagagcaacagaattttagcagctgcagaatctatgaataataccaaaaattttgttgcacagaacagaaggctaggtgcatctacccgattgaggatgccagccacagccgatggctgcaagtttgaaacggaaagaaaaccttattcgagtagaagtgattccttctctccggtgcggaagaagagattgaataatgtctctagacaaggagacagttctagttttgtgaatgcgaatatgggaggagaatcaagtccctcttctgacaaaacaagtagaaaagatgttgcttttccaatttgttctgttgatagtcactccactaaaccaaagttgccatgtttgcgagagggtgttacaaccaataatagttctgagggatgtaacgttgtttcatttacatttaaatctgcaatgaagcagaaagctggcactcatgcagaagtcacaaaaaggaagtctcagaattactcaagtgttgatgctactcgggggagatccttctttaaaggaaatgatgaagcaccatgtttgcataaatcctttcctttgaaaggggacattttaggagcacttctggagcaaaagctaaaggaattgactagtgaagaagagttcggagaagggggcgctgcacctagaaaaagcactgcaacgatccttcaggagctaataacggctttaaatgaagagaaacaatttcatctggacagttcgcccgttagacctagcaggaaagaagatttgtgtgatgatggtgatgtatcttctagaaatacttgcatgaatttccaggccataccagattcagcagcaacagatttagttgggaattcacttgatcaccatagtccgggatgtgttcttgaagctgccttttcaactgacagctacctctccagcagtcccaatagtagctcaaaggacaaagtgcttgctggatcagtggactctattgatgatgaaccactctttccagaacctgatagagatctttcggattgtgagacctcattatccaccaggagttgcagagcactgatcactgaccattttaacaacgtttctggattgctaagcaagattgatcagttaaaaggaagcaaactcagttatgcaaaagaggtcattttgaatactgaactcatatttagaactacacctcaacagcaggctctacctgtagaggatgggttctctgtgagccattttctcctcaatgaacttgaaatgctatcgagtcttctgtggatgactttcagtcagctgcttggctgtaacgacccaaaacaaatgaatcagcttaaaggattcgcctttgattgtctattagagtacctagactcaaaatttgctcgatactctgattctggtttcagaacctggaccaaactaccatcaagtatgaccaaagagattctgattgctgatattattgaagaggtcaaagagtggacagaatttgttggtttgatcccagacgagctaatagaatgggatatgagccattctttgggtaaatggaccgatttcgagattgaagaatttgaatgtggcactgaagttgctaggcatattctccaagaattagtagatgaagttgttttagacctctacagttttagctaa

SEQ ID NO: 59 - DNA, 1710 bp, Artificial Sequence
  TAF-2 CDS
atggctggagagaagattatagaaaaatctgaagcggttgctcctgggctgaaatctgattcctctaccaaactgaccgagaaggatttggtttcaaaaaatgatggaaaagtatctgactcggtgtcttctttgggagctgtgactggcatcaagggtgaaattgatcaaccaccagttgcagagcaaggtgcttattatccacctactagctattgcgattactactacccaggatataatgggacctataatcagttagatgatcaagcatactttaattcgggcgttcagtcagaaaatggttcccttctttattacatgcctggttataatccttatggtgctggatatatcggaggtgacggaaagcagccctatctatcgtctggatatcttcagcaacctgtctcatatggttcggattccatgccatgttattcatggggtggttcgacgtactgtgcagatatcaccaatagtgctgctcccaaatccggcaatgtcaaatcaacttttggacgaaatggttcggtgagatcaaacggttttaatccaacaaaaacgaatggttctttctcgagcaaaaactcgaccatgctttttaacccaaagaatcgaccgtctactgccatatcaaatccaccaaagtctatccatcaagctcagccttttaatcctgcgaacaagtctgatgtccagtccggaggcctgacaaaggggtatcatatggttggggacttcccatcatacagcagtcaaaatcaagggtttttcatgccttatgatcccattcactatcaaacaaacagtagattgtggaatgggaactataggggtaaaccacggggaaatttcaccagaaatggtgtgtttgaggcatcgaatgagttacctcgtggtccccgtgccaacagcaggagcgccccttcaaaaccatctgctgaggaggatcagcttgagccaacaattcagagggagaagtataacaaggaggattttaagactcagtatgataatgcaaagttttacattatcaagtcgtacagtgaagatgatattcacaagtgtgtcaaatatgctgtatggtcaagtactcctaatggaaacaagaaattggacactgcgttccttgatgctgagggtaaagcaagtggaactgattcaagctgtccagtgttcctcttcttttcagtaaatggaagtggacagtttttaggtgtagctgagatggttgggcaggttgacttcaacagaaacatggacttttggcagcttgataagtggagtgggttcttcccagtgaagtggcacatagttaaagatgtccctaacacacagttcaggcacatcatcctcaaaaacaatgataatagacctgtaacctatagcagagatactcaggagattggtttgaaggaaggtttggaaatgcttaacatacttaagaactactcggagaagacatctatattggatgatttcaatttctatgagaagcgtgagaaagtgctcaaggctaaaaggagttcaaaaccagctattcaagctgatgtatttgagaaagctgattctgttaggcaattcaaaggaggagataaggtacgcgaagaggagctaaagagcaactcgactgatccaactgcatctctcgtttctcttgccaaaaatctatcgattaattcgaggccattcaaaagtagtgtctga

SEQ ID NO: 60 - DNA, 1428 bp, Artificial Sequence
  Adenylyl cyclase-associated CDS
atggaggagaaattggtacagcgattggaatcggcggtggcgcggctggaggcgttatcagccaccggcttccgttccggcggttccgtcgtggcaggtggcgatggtacggcggttttagatccgtcgattattgcatttgacgatctacggtcgcagtttctttcgaaggttttgagtgctgcagagaagatcggaggacaagttttggatgttagtaagattgttgaggaggcttttgaagctcagagagaacttctcattaaaatcaaggagactaagaaaccagacaactcaggtttggttgaatttctcaaaccattgaatgatgtgatcgtgaaagctacaaaaatgactgaaggacgccggtctgatttcttcaaccacctgaaatcggctgttgatagtctatcggctctagcatggattgcctacattggaaaagactgcggaatgagcatgcctattgcattcgtggaagaaagttggcagatggctgaattttataataacaagattcttgtggagtttaaaaacaaagacccaaatcatgttgaatgggcaaaagctttgaaagaactttacctccctggattgagagattatgttaagagtcactatccattaggtcctgtgtggagcgctacagggaaacctgctgtatctgcaccttcgaaagctccttcaccaagtgctcctgctcctccagttccccctccagcttctctcttcagctctgaatctcctcaggcttcatcatcgcgccccaagcaagggatgtctgctgtctttgatgaaattaattcgggaaagccagtgacttctggattgagaaaagtaacagatgacatgaagacaaagaaccgtttcgacagaaccggcgttgttaatgctggtgataaggaagctcgcatgagctcaccccctgtctctaaaactggacctccaaaattggagcttcagatgggccgtaaatgggtggttgagaatcaagttggacaaaagaacctagttattgatgattgcgatacaaagcaatcagtatatgtctatgggtgcaaagattccgttctgcagatcaaaggaaaagtcaataacctcacaattgacaaatgcactaagatgggaattgtattcgcgggtgttgtggcagcttgtgaggttgtcaattgcaacagtgtagaggtgcaatgtcagggctcggctcctacaatatcaatcgacaatacaaatggatgccagttatacttgaacaaagattctttggagggttctattaccacagctaagtcaagtgaaatcaatgttttggttcctggtgcagggcctgatgatgattggggtgagcatgctttgccacagcagtatgctcatgaatacaaggacggacactttgtgactactcctgtctcccactctggagcttaa

SEQ ID NO: 61 - DNA, 1419 bp, Artificial Sequence
  Adenylyl cyclase-associated CDS
atggatgagaaattgatacagagattggagtccgccgtaatacggctggaggcgctgtcagtcggtggcggagcttcagttggagatggtgtagctgcggcagctttagatccatctattattgcctttgacgatctgaggtcacagttcgtaggcagagtccttggtgctgcagagaagattggtggacaagttttggacgtgactaagattgttgaagaggcttttgaagctcagagagaacttcttatcaaaatcaaggaaactcagaaacctagcatgtctggtttgcctgaatttctgaaacctctgaatgatgtgattctgaaagctacaaaaatgacagaaggatggcgacttgatttcttcaaccacttgaagtctgctgttgatagtctaatagccctggcatggattgcttacactggaaaagattgtggtatgagtatgcctattgcacacgtggaagaaagttggcagatggctgaattttacaataacaaggtccttgtggagttcagaaacaaagacccaaatcatattgaatgggcaaaagctttgaaagagctttatctccctggcttgtgggattatgttaagagtcactatccactgggccctgtatggagtgctacaggtaaagttgctgtatctgcaccatcaaaagctcctttgccaacaagtcgtcccatgccgcctcccctgccgccagcttctctattcagctctggatctttccaggcttcatcatcacgcccgaagaaagggatggcagctgtttttgatgaaattaattcggggaagccagttaccaccggattaagaaaggtgaccgatgatatgaagacaaagaaccgagcagacagaaccggtgtcattagtgccggagaaaaggaaggtcgccttagctcaccctctttctctaaagctggacctccaaaactggagcttcagatgggccgtaaatggatggttgagaatcaaataggaagaaagaatctagtcattgatgattgcgatgcaaaacaatctgtctatatttttgggtgcaaagattcagttctgcagatccaagggaaagtcaacaacataacaattgataagtgcactaaaatgggagttgtattcacggatgtcgtggcagcttgtgaggttgtcaactgcaatggtgtggagatgcaatgtcagggttcagcaccaacaatttcagttgataatacaactggatgtcaattatacttgggcaaagattcttcggagacttccattacaacagctaagtcaagtgaaatcaatgttttggttcctggtgcagggcctgatagtgattggggtgagcacgctttgccgcagcagttttctcatgtatataagaatggccagtttgtgactacatctgtctcccattcaggaggttaa

SEQ ID NO: 62 - DNA, 1470 bp, Artificial Sequence
  PMT CDS
atggctccaggaataggacaagagcgtgagattcaaaagagttattggatcgagaaaactgctggacttaaattggaggcaatgatgcatgtgcatgatcttgaatcatctgatcttgataaagaggataggcatgaggtgctttcactgctcccgtcatatgaagggaaatccgtgttggaattgggtgctggtattggtcgtttcacaggagacttagccaagaaggctggggagctcgtagcagtggattttattgaaggagtgattaaggagaatgaaagcatcagcgggcaccacaagaatgtcaagtttaagtgtgctgatgtgacttcaccagatttgacgttttcacctgaatctgtggacttgatattctctaactggctactgatgtatctttctgatgaagaggtgcaggaccttgcggagagaatgatgacatggttgaaagttggtggatatatattttttagagagacatgcttccatcagtccggagacaacaagggaaagaacaacccaactcactatcgggaacctagattctatacaaaggttttccaagaatgtaatgctggaaaatcatatgaactttctctcgtcggttataagtgcatggaaacttatgtaagaaacaaaaggaatcaaaatgagatttgctggatatggcagaaggttcgttctgatgatgacaggggattccagcatttcttggacactgttcagtacaagtctaatggcatactgcgatatgaacgtgtctttgggaaagactttgtgagcacaggtggaatcgataccaccaaagaattcgttgccatgttggatcttcagcctggcgaaaaagtccttgatgttggctgtggcatcggtggtggtgacttttatatggctgagaagtatgatgttcatgttctcggcattgatctctcagttaacatgatctcattgtcttttgaacgtgctattggtcgcaaatgcgcggttgaatttgaggttgctgattgcacagtgaaaacatatcctgaaggatcattcgacgtgatatacagccgggacactatcctgcacatccaggataaaccagcattattccaatctttctacaagtggctgaagcccggaggcagagtcctcataagtgactattgcaaaaaggcagggccagcatcagaagaatttgcagcgtacatcaaacaaagaggttacgatttacatgatgttgaagcatatggacagatgcttagagatgctggtttcaatgaagttattgctgaggatcgaactgagttgttcatgaaagttctccagaaagagttggatattgtggagaaggaaagagagtcatttatccaggagttttctgaacaagactataatgatatagttggaggttggaaggccaagctagtgaggagttcatctggtgaacagagatggggtttattcattgccaagaaaaattga

SEQ ID NO: 63 - DNA, 1476 bp, Artificial Sequence
  PMT CDS
atggatgttgcttcaggacaagagcgtgaggttcagaagagttattggattgagcatactgctgaacttactgttgaggccatgatgctcgactctaaagcagccgatctagacaaagaggagaggcctgaggtgctctctctgcttccggcatatgaagggaaaactgtgttggaactgggtgctggtattggccgtttcactggtgaattagccaagaaagctggacagcttatagcattggactttattgaaggcgcaattaagaagaatgaaagcataaatgggtgccataagaatgtcaagttcatgtgtgctgatgtgacttctccagatttgaatttttcaccggaatcggtggacttgatattttctaattggctgctgatgtatctttctgatgaggaggttcaggatcttgctaagagaatggttaaatggttgaaagtcggtggttacatatttttcagagagtcgtgcttccatcaatcaggagaccataagcgaaagaacaacccaacccactatcgagatcctagcttttatacaaaggttttcagagaatgtcatgtaaatgctggtgatggaaaatcatttgaactttctcttggcggttgcaagtgcatcggtgcttatgtgaggaacaaaaagaatcaaaatcagatttgctggtcgtggcagaaggttggttctgagaatgacatggaatttcagcgcttcttggatactgttcagtacaagtgtagtggcatactacgctatgagcgagtctttggacaaggttttgtgagcacaggaggacttgaaactaccaaagaatttgtagccatgttggatcttcagcctggccagaaagtccttgatgttggctgtggcattggaggaggtgacttctacatggcagaaaagtacgatgttcacgtcgttggcattgacctgtctatcaacatgatatcatttgctcttgagcgtgctattggtctcaagtgtgctgttgaatttgaggttgctgattgcaccaagaaaacatatcctgttggtacatttgatgtcatatacagtcgggatactatccttcacatccaggacaaacctgcactcttcagatctttctacaagtggctgaaaccaggaggcaaagtccttataagtgattactgcaaaagagccggaccagcatcagaagaatttgcaggttacattaagcaaaggggatatgatttacatgatgttgaagcatatgggcagatgctcagagatgcaggttttcatgatgttgtggccgaggatcgtactgaacagttcattggggttctgcaaaaggagttggatactgtggagaagggaagagagtcatttatccatgagttctctgaacaagactataatgaaatagttggaggttggaaagccaagctaatcaggagttcatctggtgagcagaggtggggcttgttcgttgccaagaagaactga

SEQ ID NO: 64 - DNA, 816 bp, Artificial Sequence
  PMT CDS
atgctatgctggctatggcagaaagttaattctgaggatgacaggggattccagcgtttcctggacaacgcgcaatacaagtgtagtggcatactgcgatatgaacgtgtctttggagaaggttatgtgagcacaggaggaattgataccacaaaagaatttgtctccatgttggatcttcaacctggccaaaaagtccttgatgttggctgtggaataggtggaggtgacttttacatggctgagaattatgatgttcatgttgttcccattgacctctcaattaacatgatatctttcgctcttgagcgtgcaattggtctcaaatgtgccgtcaaatttgaggttgctgattgtacaaagaaaacgtatcctgatggcacatttgatgtgatatacagtcgagacactatccttcatatccaagacaaacttgcgttattcagatctttctacaggtggctgaaaccaggaggcaaagtcctcataagcgactactgcaaaagaccaggacctgcatcggaagatttttcaggctatattaagcgaaggggttatgatttacattatgttgaagcatatggcctgatgctcagagaggcgggtttcgatgaagttattgccaaggatcgaactgaacagttcattaatgttctccggaaggagttgtatactgtggagaaggaacgagattcatttttccaggaattctcagaacaaggctacaatgaaatagttggaggttggaacgccaagctattgaggagttcatctggtgaacagaggtggggattgttcattgccaagaagaagtga

SEQ ID NO: 65 - DNA, 2193 bp, Artificial Sequence
  DnaJ domain-containing CDS
atggagtgcaataaagacgaggccctcagagcaaaaataattgcagagcggaagtttgaacaaaaggattatgctggtgcaaagaaatttgccttgaaagctcaggctttgtatccggggcttgacgctctagcccagatgttaacaacacttgatatctacatcgctgctgaaaataaaataagtggggaagtggattggtatggggtacttggtgtgagcccgtcaactgatgatgaaacagtgaggaaacagtacaggaagctagctctcattctccaccccgataaaaacaaatctgttggtgctgaaggtgcatttaaacttctctctgaggcctggagcttgttgagtgataaatccaagaggttggcatataaccagaggaggagttcaaaaggattccagcagaaagctccagtacactcgggtggtccgtcagcacctccacgaaatgggtttcataattttactagtaagacttcgaagactcagaaaaatgcttctcgggtgccctcttcatcagttaattcttcagccaaccaaagaagtgatactttctggaccatttgccaccgatgcaagatgcattatgagtatttgaaaatttatcttaaccacactcttctgtgccccaactgtcatgaagcttttatggccacagaaacagccccaccgttcaatcatgcaaaatcatccaattctacgcgtcagtggcatcagaatgctgggaatcatgcacctaatggaaatcaattcccaataggaagaaatgctagtgctggaaaaacatcaggatcagcaccagcaagttctaatactgcgaattattcgaactttcagcaggactcattttccagaatggctggtgttggtagctcggatccttccattgcagcaaaagctgcaaatgttgttcagcaggcacatgagaaaatgaagagagaacgtgatgattcacagactagacagcctcctcttaaacagagaaagcttgatgacaatggaatccgttatggatccaatatacctcactatgcagaaagggcttatggtttctcttctagcaagtttaacagtacaagggagctgacaccacttgaaaaccggaatatgctgatgggaaaagctcggaaagagatactcagtaagttgaatgaatggagatcgcagccgcaagatgcacaaaaaaataaggtgaaagagggcaaaaaagaaaagcagagggctgctaatgttcttggccaaaatgtgaatgggaatgtcgagtcatcagctatgaagggggtaaagaaagatgttaatgcttcagctaatgatgcaaaacaagaggatctactgccacaatcaatgaatgtaccagatcctgattttcacaattttgaccaggataggagcgaaagttgtttcggagacaatgaagtctgggctgcatatgatgctgatgatgggatgccccgtttctacgctctgattagcaaagtcgtctcaagggagccatttaaagtgaggcttagttggcttaattcaaagacaaacagtgaatttggtccaatggaatgggtagcttcaggtttctacaagactagtggtgaatttaggattggcagatacgaaacgagtaagtctgtgaattccttctcccacaaggttcggtggtcaaagggccctcgtggatctgttctcatatttcccatgaagggggaggtttgggccctctacagacattggtctcctgactggaatcagaatacacctgatgatgtcatacacaagtatgacatggtcctagttcttgatgactacaatgaggagcaaggaatttcagtagctcctctcgtcaaagttgctggttttaaaacggtctttcgtccagatttgaattcggagaaggtgatgagaatcaccagagaagagatgtttcgtttctctcatcgggtcccaagccacttgcttacaggtgaagaagctcaaaatgctccaaagggttgccaggagcttgatccagctgctaccccattggagcttcttcagacattaccagaaactaatggggtgtcagccatgcagaatgacaaagattttaatggactttcaccacagaatgttcaggagactaaaactagagagactgctgatcatactctcaactccagtgaagacgggatggtaaacggtgaagaagctccatga

SEQ ID NO: 66 - DNA, 1245 bp, Artificial Sequence
  Elongation factor 1-gamma 1 (eEF1B)
atggctttgattttacattcaacaagtaacaacaaaaatgccgcaaagggactcattgcggctgagtacacaggtgtgaaagttgaacttgcaaaggatttccagatgggtgtgtcaaacaagacacctgaatttctcgagatgaatccaattggaaaggttcctgtgcttcaaacacctgatggacctgtttttgagagcaatgctattgcacgttatgttaccaaaacgaagcccgataatcttctttttggctcttcattgattgaatatgctcaaattgaacaatggaatgatttttctgccactgaagttgatgcaaacattgcacgttggctgtacccacgccttggctatgccgtatacattcctccagctgaggaagctgcggtagctgcattaaagagagctcttggtgctttgaacacccatctcgcatccaacacatacttggttggacattcaatcacattggctgacattattatggtctgcaacttgagcattggttttggggtgataatgaccaagagctttaccaaagaattcccacatgtagagagatacttctggactgtggttaatcagccaaatttctgcaagatattgggtgaggttaaacaagctgaatctatcccagctccgccatccaagaagcccgcaccggcgacagaaaagcccaaggctaaggaggagccaaagaaagaggttaaggaagaacctaagcctgcagaggaggaagcagcacccaagcctaagccaaagaatcctcttgatctcttgcctccaagtccgatgattctggatgattggaagaggctttactccaacaccaagaccaacttccgtgaggttgctgttaaaggtttctgggacatgtatgaccctgaaggatattctctctggttttgcgattacaagtacaatgatgagaacacagtttcgtttgtaaccttgaacaaggttggtggttttctgcaaaggatggatctggtgcgcaagtatgcttttggtaagatgttgattgttggttctgagcccccattcaaggtgcaaggcttgtggcttttccgtggaaaggaaattcccaagttcgttatggatgaagtctacgacatggagctctatgaatggaagcaagtagacatcaacgatgaagcccagaaggaacgtgttagccaaatgattgaagaccatgagccttttgagggacaggctctgttggatgcaaagtgcttcaagtaa

SEQ ID NO: 67 - DNA, 5724 bp, Artificial Sequence
  TPR-like superfamily CDS
atggcaccaagcaagaatggtcgtggcaaaactaagggagacaagaagaagaaagaagagaaggttcttcccgttgtaatggatataacgataaaccttccggatgagactcaagttattttaaagggaatatctacggatagaattattgacgttcgtcgattactatctgtgaacacaacaacttgtaatattaccaatttctcactgtctcatgagttaaggggtccacgtttaaaagaaacagtggacgtttccgcactgaagccctgcctcctgactctcatagaagaggactacgatgaagaaagcgccacggcgcatgttataaggctgctggatatcgttgcatgtacgacgagctttgggccgtcggggactaatggcaaggacttgaaaactgagtctagtaagaatgcgcggggtgcgcaggatagtaagggcgccaaaaaatcaagcaaggttcaggcaaatgataagtcatcgtcgccgccacaaacgccaactccggcggcggcgtctcaacaggcgggtaaagatgcagcgtcagtggatgttgatggagagatgagcaatacgtgccctaagattggaagcttctatgagttcttctcgctttctcatctcactcctccgcttcagttcataagaagagcgacaagacagcaagatggtgaagttttgccagatgatcatcttttcactcttgaagtgaaactttgtaatggaaagctggttatagttgaagcttgcaagaaaggattttataactttgggaagcaggggattctttgtcacaatcttgttgatttgttgagacaagtcagtagagcatttgacaatgcttacgatgagctcatgaaagcattctcagagcgtaataagtttgggaatcttccctacggattcagagccaacacatggcttataccacctgtggcagcacaattgccagctatctttccacctctacctgtggaggatgaaaactggggagcaaatggaggtgggcttggccgagatggcaaatttgatttgttaccttatgccaatgaatttttgaatgttgcatccatgccttgtaagacaacagaggagaggcagatacgagacaggaaggcttttcttcttcatagtttatttgttgatgtcgccattttacgagccatttcagctgtaaagcatgtcatggagaaagttaaaccagctcattgtaattcgaatggagaaatcattttgactgagtcagttggggatttgagcatatttgttaccaaagatgcttcaaatgctagcagcaaagtagataccaaaattgatggatttcaagcaactggaatagctatgaagaatctgatggaaagaaatttgctgaaggggataactgctgatgaaaatactgctgcccatgatgttgctactttaggtgttttgaatgtaaggcattgtggttatattgcaactgtaaaagttcaaggaaaagaaaatgacaaagtgggcagcccactgcaaagcatggaacttcctgatcagcctgatggtggtgcaaatgccctcaatatcaacagtttgcgtttactccttcacaagaaagtggtcaacaaggtaatgcattcaaaaccttcagattctgaagagacaaactgctctcaggcatttgtaaagagaatactagaagagagtcttaccaaacttgaagaagagaaaatagaaggtgactctttcatcagatgggaacttggtgcatgctggatacaacacttacaagatcagaagaaatcagaaaaggacaaaaagaaccctgttgagaagacaaaaaatgagatgaaggttgagggacttggaataccactcaagtcccttaagaacagaaagaagagctcagatggtgctaacacggaatcccagtctgacaccttcaaatctatcgcagatggtgttcaaaggggatcagaaaaaactgtcctgcagtctggggagtcgcagtttgagactgatacggatcaaaatcaggtcgtcctcaaggcattgttgtctgatgctggttttactaggttgaaagagtcagagactggacttcaccttaagtctttggaagagctgattgttctgtcacagaagtattacaacgaagttgccctgccaaagctggtggctgattttggctctttggaactctcaccggtagatggtcgaaccttaactgatttcatgcatacacggggtctacgtatgcgttctcttggacaagtagttaaactttctgagaagttgtcacatgtgcaatctctttgtatacatgagatgatagttcgagcttttaaacatattctgcaagcagttattgcatcggttgttgatattgaggatatggctgcaataattgctgctgctttgaatatgatgcttggggtacctgaaaatgatgatgcaaatgagttaggtgttgattctttgatctggatatggctggaattatttttgaagaagcgatatgaatgggatgttggcagcctaaactacaaagatgtgaggaaatttgcgatcctccgtggtttatgccataaggtgggaattgaactggttccaagagattatgatatgagttccccaagtccttttcagaaagtagacattgtcagcctagtaccagtgcataagcaagctgcttgctcttctgcagacggaaggcagcttttggagtcgtccaaaacagctctggataagggaaaacttgaagatgctgtcagttatgggactaaggctcttgccaagctggtcgcagtatgtggtccatatcatcgaatgactgctggagcttatagtcttcttgctgttgttctgtatcacaccggtgattttaatcaggccacaatttatcagcagaaggccttggacataaatgagagagagttgggcctcgatcacccagacacaatgaaaagttatggtgatcttgcagttttctattaccgacttcaacacacagagttggctctcaagtatgtaaaacgagctctttatttgttgcatctcacatgtggcccctcgcatccaaacactgcagcaacatatataaatgtggctatgatggaggaagggctcggtaatgtgcatgttgccctcagatatctccataaagctttgaagtgtaaccaaaagttacttggtccagaccatattcagacagctgcaagttatcatgctatagcaattgcactctctttgatggaagcttatcctttgagtgttcagcatgagcaaacaaccttgcagatacttcgagcaaagcttggtccagatgatcttcgcacacaggatgctgctgcatggctcgagtattttgagtcaaaggcgtttgaacaacaagaagctgctcgaaatggaactaagaagcctgatgcatcaatagctagcaagggccatttgagtgtgtcagatttgctcgactacatcaatccaagtcctgatgccaaagggagagatgttggatcaaaaagaaaaggttttgtctcaaaggctcttttttctcaggtgaagggaaaatctgagcaaagcaatgtttccataccaaactctgacactcctaaagatgtccccaaagaagaaacagatgagaagaaacaacttatcgaagatcatacagatcccaagatgcatatggaacccgttgacacagtaattgaatccaatcataatggagatggaagaattgctgagaacaaacccatccaatctggacccttgctgaaggaaactttaattgagaagtctacagtccatgaagtgttatctgaaccttctgctgaagcagaagatggatggcagccagtgcagagaccaaggtcaggtggtttctatggacgaagacgaaggcagaggcgtcaaaccatcagcaaagtcattggttaccagaaaaaggacccagtttctgatgttgatcatgctaaattgaagaataactatcaagctagtaaatattatgtcttaaagaaacggacatcaccaggaagttatgcagattattacatagcaaaaagtcaaactcctggtaccaaacttggtcgaagagtcataaaagctgtagcctaccgcgtaaagtctgtatcaccttctgtcagagatgctgttcctgagatttccacaactggaggagatttaactacttcatcagagcaggtccaagtttctgtaacaaaagaggttggatcagtagcaaagagaagttctatagtaaaccttggaaaatctccttcctataaagaagtagcacttgccccgccaggtaccatctctatgttgcaggagagagtttctgaaggtgaaattcctgataatcaagacattacaaaacttgaagaggagagcaacggagcagaaacaaattccaaaacaatgaaaagtgatgcagaatccgtggagaaagagaacattcaggatcttgttgcagattctgctgatcatgttaaaagtgaaacagtagctactgacaaaaaagaagaaattcaaatgagtgatcttgacggtggtgaaatttcagatgtgatatctgcaaatacatctattcaacccggccatgttgatgttagtccagtggaacaggttagtgtcgagactcataatgtccctccttctgacaattctcccaaagtggatccctgtgaaaaggactcatcaagccatttaaatccaacctgtatctcgaatatgaccttgcaagatatggatcatctgaaggtaaaatctgcatcatctcatacaagtgatgcaagtcgagaattgtctagaaagctatccgcatcagcaacaccattcagcccttccccagccgttccccgcgtagcaccattacctatgaacattaatctcccttctcctcctggaatacgaccacctgttggcccttggccagtgaacatgtctcttcatcaaggaccaccgaccatcttgcccaatccaatgtgctcctcccctcaccacctgtacccttcacctccacacaccccaaacatgatgcacccattgcgctttatctaccctccgtattctcaaccccagacgatacctccaagtactttccccatgaatagcagcactttccatccgaatcattatgcttggcaatgcaacatagctcctaatgcatcagagtatgttcctgccacagtttggcctggctgccacccagtcgagttttctatctcaccacctgtaattgagtctataactgactcaatatctgctgctaaggagctatctgacaatcctgaaagcattagtttgacaacaagcttaccagtagatctgaacaccggagatgaagtcaaagaagatgaaaatcttccagtatcggaaatggtggagagcttagctgctgttggatcagaaaaagagagagcaagcaacacttcagattcacattttgttaccttctctagtgatcaatcaaaagagggaagtggatcaaatgagaaggctggaagttgcagtgacaattatgtgcaaagaaatcttgtggagacggatgatgagaagaccttcaacattttggtacggggccggaggaaccgcaaacaaactctaagaatgccaataagtttgctcaagagaccatattcttctcagcccttcaaagctgtatatagtagggttataagggagactgaggttcccaggtctaccagctttgatccacatgaacattgcataacgactgctacttga

SEQ ID NO: 68 - DNA, 789 bp, Artificial Sequence
  XRI1-like CDS
atgggtgaccttcactcaattgcttacaacaacaataatctccatagcttatcttccctaggttgtgacttccatggccttgaagttttcaacaatgacatatctccatttatggagagcactccaccatttttatcaaatcttgattgtgacttatcaagtggatatctacaagatgcattattcaaattcaactcaaaaagaagacgtttattattatttgatgatgatgatgaagagaaggagaattatcaaattaatgattcaaataattccattaagaatttgtggagttccacaatggaccaacaattttctgaggattatgattgttttagccaaataaccaagtgtgatagcttttctggtgatcccatgagcaaaatgagtgaagaatattcaaaggaggaagcaatatcagaaaattattattattattcatcttcaccaacatcatcatctcatcataataatattaatcaaaaacaattaccccaacaatatggaggagttgatcaaaagagaagcaagaaaaggatggttggaaaaattgtgtgtccatttgggctagttaagccaggagggcaagaaggtgatgtgacattaaatgacatcaatgagaggattttgatgaggccaacccggcccgttaggcatccggtcggggactttgcatgtcgcccgaccgtatcaccagccggaccagggttgtccggtaagaaagtagtcgcgctcactaaaattcatactcaagggagagggacaatcacgattataaggactcgaggg

SEQ ID NO: 69 - DNA, 801 bp, Artificial Sequence
  ToBRFV movement protein CDS
atggctcttgttaagggtaaagtcaatattaatgagttcatagacttgtcaaaatcagaaaaatttcttccgtctatgttcacacctgttaagagtgtcatgatctccaaggttgataagatattggttcatgaagatgaatctttgtccgaagtcaatttactcaaaggtgtaaaactcattgatggtggctatgtacatcttgctggtcttgtggtgacaggtgaatggaatttgccagataattgtcgtggtggtgtcagtgtctgtttggtcgataagagaatggagagagcggacgaggcaactcttgcttcatactataccgcagcggctaagaaaaggtttcagttcaaagtcgttccaaattacaacatcactaccaaggacgcagaaaaggcagtttggcaagtactagttaatattagaaatgttaaaattgctgcgggttactgtccgctgtcattagaatttgtgtcagtgtgtattgtttataaaaatattataaaactcggtttgagagagaaaattacgagcgtcacggatggagggcccatggaactatcagaagaagttgttgatgagttcatggaagaagtcccgatgtctgtaaggcttgcaaaatttcgttcgaagaccggaaaaaagtttagtagtaaaagtgagaataatagtggtaataataggccgaaaccagacaaaaaccaaaggaaggaaaagggtttaaaagttagggttgagaaggataatttaattgataatgaattggagacttacgtcgccgattcagattcgtattaa